European Patent Application EP 4 488 292 A1, published January 8, 2025. Title: 神経変性疾患の治療剤. Applicant: 帝人ファーマ株式会社. Application JP. The sequence listing filed with the application follows.

SEQUENCE LISTING (302 sequences)

SEQ ID NO: 1 - protein, 8 aa, Artificial Sequence
GYAFSNHL

SEQ ID NO: 2 - DNA, 24 bp, Artificial Sequence
  source 1..24: mol_type = other DNA
ggctacgccttcagcaaccacctg

SEQ ID NO: 3 - protein, 8 aa, Artificial Sequence
INPGSGGT

SEQ ID NO: 4 - DNA, 24 bp, Artificial Sequence
  source 1..24: mol_type = other DNA
atcaaccctggcagcggcggcacc

SEQ ID NO: 5 - protein, 12 aa, Artificial Sequence
ARGANWDVGFAY

SEQ ID NO: 6 - DNA, 36 bp, Artificial Sequence
  source 1..36: mol_type = other DNA
gctagaggcgctaattgggacgtggggttcgcgtat

SEQ ID NO: 7 - protein, 6 aa, Artificial Sequence
QDIVKN

SEQ ID NO: 8 - DNA, 18 bp, Artificial Sequence
  source 1..18: mol_type = other DNA
caagacatcgtgaagaac

SEQ ID NO: 9-10 - skipped (2 entries)

SEQ ID NO: 11 - protein, 9 aa, Artificial Sequence
LQFHEFPRT

SEQ ID NO: 12 - DNA, 27 bp, Artificial Sequence
  source 1..27: mol_type = other DNA
ctgcagttccacgagttccctagaacc

SEQ ID NO: 13 - protein, 119 aa, Artificial Sequence
QVQLQQSGAELVRPGTSVKVSCKASGYAFSNHLIEWVKQRPGQGLEWIGVINPGSGGTNYIEKFKGKATLTADKSSSTAYMQLSSLTSDDSAVYFCARGANWDVGFAYWGQGTLVTVSA

SEQ ID NO: 14 - DNA, 357 bp, Artificial Sequence
  source 1..357: mol_type = other DNA
caagtgcagctgcagcaatctggcgccgagctggtgagacctggcacaagcgtgaaggtgagctgcaaggctagcggctacgccttcagcaaccacctgatcgagtgggtgaagcagagacctggccaaggcctggagtggatcggcgtgatcaaccctggcagcggcggcaccaactacatcgagaagttcaagggcaaggccaccctgaccgccgacaagagcagcagcaccgcctacatgcagctgagcagcctgacaagcgacgacagcgccgtgtacttctgcgctagaggcgctaattgggacgtggggttcgcgtattggggccaaggcaccctggtgaccgtgagcgcc

SEQ ID NO: 15 - protein, 107 aa, Artificial Sequence
EIQMTQSPSSMSASLGDRITITCQATQDIVKNLNWYQQKPGKPPSFLIYYATELAEGVPSRFSGSGSGSDFSLTISNLESEDFADYYCLQFHEFPRTFGGGTKLEIK

SEQ ID NO: 16 - DNA, 321 bp, Artificial Sequence
  source 1..321: mol_type = other DNA
gagattcagatgacacagagccctagcagcatgagcgctagcctgggcgacagaatcaccatcacctgccaagccacccaagacatcgtgaagaacctgaactggtatcagcagaagcctggcaagcctcctagcttcctgatctactacgccaccgagctggccgagggcgtgcctagcagattcagcggcagcggcagcggcagcgacttcagcctgaccatcagcaacctggagagcgaggacttcgccgactactactgcctgcagttccacgagttccctagaaccttcggcggcggcaccaagctggagatcaag

SEQ ID NO: 17 - protein, 8 aa, Artificial Sequence
GYTFTDNW

SEQ ID NO: 18 - DNA, 24 bp, Artificial Sequence
  source 1..24: mol_type = other DNA
ggctacaccttcaccgacaactgg

SEQ ID NO: 19 - protein, 8 aa, Artificial Sequence
IDPSDSFT

SEQ ID NO: 20 - DNA, 24 bp, Artificial Sequence
  source 1..24: mol_type = other DNA
atcgaccctagcgacagcttcacc

SEQ ID NO: 21 - protein, 15 aa, Artificial Sequence
TRSGYYGSPKLGGDY

SEQ ID NO: 22 - DNA, 45 bp, Artificial Sequence
  source 1..45: mol_type = other DNA
acaagaagcggctactatggctcccctaaattgggcggcgactac

SEQ ID NO: 23 - protein, 5 aa, Artificial Sequence
SSISY

SEQ ID NO: 24 - DNA, 15 bp, Artificial Sequence
  source 1..15: mol_type = other DNA
agcagcatcagctac

SEQ ID NO: 25-26 - skipped (2 entries)

SEQ ID NO: 27 - protein, 9 aa, Artificial Sequence
HQWNSYPCT

SEQ ID NO: 28 - DNA, 27 bp, Artificial Sequence
  source 1..27: mol_type = other DNA
catcagtggaacagctacccttgcacc

SEQ ID NO: 29 - protein, 122 aa, Artificial Sequence
QVQLQQPGAEIVRPGASVKLSCKASGYTFTDNWMGWVKQRPGQGLEWIGAIDPSDSFTNYNQNFKGKATLTVDTSSSTAYMQLSSLTSEDSAVYFCTRSGYYGSPKLGGDYWGQGTTLTVSS

SEQ ID NO: 30 - DNA, 366 bp, Artificial Sequence
  source 1..366: mol_type = other DNA
caagtgcagctgcagcagcctggcgccgagatcgtgagacctggcgctagcgtgaagctgagctgcaaggctagcggctacaccttcaccgacaactggatgggctgggtgaagcagagacctggccaaggcctggagtggatcggcgccatcgaccctagcgacagcttcaccaactacaatcagaacttcaagggcaaggcgacgttaaccgtcgacacaagcagcagcaccgcctacatgcagctgagcagcctgacaagcgaggacagcgccgtgtacttctgcacaagaagcggctactatggctcccctaaattgggcggcgactactggggccaaggcaccacactgacggttagctcc

SEQ ID NO: 31 - protein, 106 aa, Artificial Sequence
QIVLTQSPAIMSASLGEEITLTCSASSSISYMHWYQQKSGTSPKLLIYSTSNLASGVPSRFSGSGSGTFYSLTISSVEAEDAADYYCHQWNSYPCTFGGGTKLEIK

SEQ ID NO: 32 - DNA, 318 bp, Artificial Sequence
  source 1..318: mol_type = other DNA
cagatcgtgctgacacagagccctgccatcatgagcgctagcctgggcgaggagatcaccctgacctgcagcgctagcagcagcatcagctacatgcactggtatcagcagaagagcggtacaagccctaagctgctgatctacagcacaagcaacctggctagcggcgtgcctagcagattcagcggcagcggcagcggcaccttctacagcctgaccatcagcagcgtggaggccgaggacgccgccgactactactgccatcagtggaacagctacccttgcaccttcggcggcggcaccaagctggagatcaag

SEQ ID NO: 33 - protein, 8 aa, Artificial Sequence
GYTFTDYW

SEQ ID NO: 34 - DNA, 24 bp, Artificial Sequence
  source 1..24: mol_type = other DNA
ggctacaccttcaccgactactgg

SEQ ID NO: 35 - protein, 8 aa, Artificial Sequence
IDPSDSYT

SEQ ID NO: 36 - DNA, 24 bp, Artificial Sequence
  source 1..24: mol_type = other DNA
atcgaccctagcgacagctacacc

SEQ ID NO: 37 - protein, 15 aa, Artificial Sequence
ARSGYYGSPKLGGDY

SEQ ID NO: 38 - DNA, 45 bp, Artificial Sequence
  source 1..45: mol_type = other DNA
gctagaagcggctactatggctcccctaaattgggcggcgactac

SEQ ID NO: 39 - protein, 5 aa, Artificial Sequence
SSISY

SEQ ID NO: 40 - DNA, 15 bp, Artificial Sequence
  source 1..15: mol_type = other DNA
agcagcatcagctac

SEQ ID NO: 41-42 - skipped (2 entries)

SEQ ID NO: 43 - protein, 9 aa, Artificial Sequence
HQWNSYPCT

SEQ ID NO: 44 - DNA, 27 bp, Artificial Sequence
  source 1..27: mol_type = other DNA
catcagtggaacagctacccttgcacc

SEQ ID NO: 45 - protein, 122 aa, Artificial Sequence
QVQLQQPGAEIVRPGASVKLSCKASGYTFTDYWMNWVKQRPGQGLEWIGAIDPSDSYTNYNQEFNGKATLTVDTSSSTAYMQLSSLTSEDSAVYFCARSGYYGSPKLGGDYWGQGTTLTVSS

SEQ ID NO: 46 - DNA, 366 bp, Artificial Sequence
  source 1..366: mol_type = other DNA
caagtgcagctgcagcagcctggcgccgagatcgtgagacctggcgctagcgtgaagctgagctgcaaggctagcggctacaccttcaccgactactggatgaactgggtgaagcagagacctggccaaggcctggagtggatcggcgccatcgaccctagcgacagctacaccaactacaaccaagagttcaacggcaaggcgacgttaaccgtcgacacaagcagcagcaccgcctacatgcagctgagcagcctgacaagcgaggacagcgccgtgtacttctgcgctagaagcggctactatggctcccctaaattgggcggcgactactggggccaaggcaccacactgacggttagctcc

SEQ ID NO: 47 - protein, 106 aa, Artificial Sequence; identical to SEQ ID NO: 31

SEQ ID NO: 48 - DNA, 318 bp, Artificial Sequence; identical to SEQ ID NO: 32
  source 1..318: mol_type = other DNA

SEQ ID NO: 49 - protein, 8 aa, Artificial Sequence
GYTFTDCY

SEQ ID NO: 50 - DNA, 24 bp, Artificial Sequence
  source 1..24: mol_type = other DNA
gggtacacctttaccgactgctac

SEQ ID NO: 51 - protein, 8 aa, Artificial Sequence
INPNSGYT

SEQ ID NO: 52 - DNA, 24 bp, Artificial Sequence
  source 1..24: mol_type = other DNA
atcaaccccaacagtggctacacg

SEQ ID NO: 53 - protein, 16 aa, Artificial Sequence
TRGDYYTSNLYDWFAY

SEQ ID NO: 54 - DNA, 48 bp, Artificial Sequence
  source 1..48: mol_type = other DNA
acaagaggcgattactacacctccaatctctatgactggtttgcatac

SEQ ID NO: 55 - protein, 6 aa, Artificial Sequence
QTVGTV

SEQ ID NO: 56 - DNA, 18 bp, Artificial Sequence
  source 1..18: mol_type = other DNA
cagaccgtagggactgtg

SEQ ID NO: 57-58 - skipped (2 entries)

SEQ ID NO: 59 - protein, 9 aa, Artificial Sequence
LQYGSVPPT

SEQ ID NO: 60 - DNA, 27 bp, Artificial Sequence
  source 1..27: mol_type = other DNA
ctgcagtatggcagcgttccacccacc

SEQ ID NO: 61 - protein, 123 aa, Artificial Sequence
QVNLLQSGAALVKPGASVRLSCKTSGYTFTDCYIHWVRQSHGKSLEWIGFINPNSGYTFYNEKFKSKATLTVAKSTNTAYMELSRLTSEDSATYFCTRGDYYTSNLYDWFAYWGQGTLVTVSS

SEQ ID NO: 62 - DNA, 369 bp, Artificial Sequence
  source 1..369: mol_type = other DNA
caggtcaatctgctgcagtccggagctgcattggtcaaacccggagccagcgtacggctttcctgtaagacatctgggtacacctttaccgactgctacattcactgggtaaggcagtcacatgggaagagccttgagtggattggcttcatcaaccccaacagtggctacacgttctacaacgagaagttcaagtccaaagctacactgacagtggccaaaagcaccaacactgcctatatggagctgtcacgcttgacatccgaagatagtgccacatatttctgcacaagaggcgattactacacctccaatctctatgactggtttgcatactggggtcaaggcaccctggttaccgtgtcatct

SEQ ID NO: 63 - protein, 107 aa, Artificial Sequence
DTVMTQSPASMSTSVGERVTVNCKASQTVGTVVAWFQQKPGQSPKRLIYWATNRHTGVPDRFTGSGFGRDFSLTISNVEAEDLAVYYCLQYGSVPPTFGGGTKLELK

SEQ ID NO: 64 - DNA, 321 bp, Artificial Sequence
  source 1..321: mol_type = other DNA
gacacagtcatgacccaatcaccagcatccatgagcacttcagttggcgagagagtgaccgtgaactgtaaggcctctcagaccgtagggactgtggttgcctggttccagcagaaaccagggcaaagccccaaacggctgatatactgggcaacgaatcgacacactggtgtacctgaccgctttaccggcagtgggttcggaagggacttctccctcaccatttccaacgtcgaagccgaagatcttgccgtgtactattgcctgcagtatggcagcgttccacccacctttggaggaggcacaaagttggagctgaag

SEQ ID NO: 65 - protein, 8 aa, Artificial Sequence
GYTFTNHN

SEQ ID NO: 66 - DNA, 24 bp, Artificial Sequence
  source 1..24: mol_type = other DNA
ggctacacatttaccaatcacaat

SEQ ID NO: 67 - protein, 8 aa, Artificial Sequence
FYTGNGDT

SEQ ID NO: 68 - DNA, 24 bp, Artificial Sequence
  source 1..24: mol_type = other DNA
ttttatacaggaaatggtgatact

SEQ ID NO: 69 - protein, 14 aa, Artificial Sequence
ARERYDGYYIAMDY

SEQ ID NO: 70 - DNA, 42 bp, Artificial Sequence
  source 1..42: mol_type = other DNA
gcaagagaaaggtatgatggttactatattgctatggactac

SEQ ID NO: 71 - protein, 5 aa, Artificial Sequence
SSVYY

SEQ ID NO: 72 - DNA, 15 bp, Artificial Sequence
  source 1..15: mol_type = other DNA
tcgagtgtgtattac

SEQ ID NO: 73-74 - skipped (2 entries)

SEQ ID NO: 75 - protein, 10 aa, Artificial Sequence
QQWSSNPQWT

SEQ ID NO: 76 - DNA, 30 bp, Artificial Sequence
  source 1..30: mol_type = other DNA
cagcagtggagtagtaacccacagtggacg

SEQ ID NO: 77 - protein, 121 aa, Artificial Sequence
QVQLQQPGAELVKPGASVKMSCKASGYTFTNHNMHWVKQTPGQGLEWIGAFYTGNGDTSYNQKFKGKATLTADKSSSTAYIQLSSLTSEDSAVYYCARERYDGYYIAMDYWGQGTSVTVSS

SEQ ID NO: 78 - DNA, 363 bp, Artificial Sequence
  source 1..363: mol_type = other DNA
caggtacaactgcagcagcctggggctgagctggtgaagcctggggcctcagtgaagatgtcctgcaaggcttctggctacacatttaccaatcacaatatgcactgggtaaagcagacacctggacagggcctggaatggattggagctttttatacaggaaatggtgatacttcctacaatcagaagttcaagggcaaggccacattgactgcagacaaatcctccagcacagcctacatacaactcagcagcctgacatctgaggactctgcggtctattactgtgcaagagaaaggtatgatggttactatattgctatggactactggggtcaaggaacctcagtcaccgtctcctca

SEQ ID NO: 79 - protein, 107 aa, Artificial Sequence
QIVLTQSPAFMSVSPGEKVTMTCSASSSVYYMFWYQQKPRSSPKPWIYLTSKLASGVPARFSGSGSGTSYSVTISSMEAEDAATYYCQQWSSNPQWTFGGGTKLEIK

SEQ ID NO: 80 - DNA, 321 bp, Artificial Sequence
  source 1..321: mol_type = other DNA
caaattgttctcacccagtctccagcattcatgtctgtatctccaggggagaaggtcaccatgacctgcagtgccagctcgagtgtgtattacatgttctggtaccagcagaagccaagatcctcccccaaaccctggatttatctcacatccaagctggcttctggagtccctgctcgcttcagtggcagtgggtctgggacctcttactctgtcacaatcagcagcatggaggctgaagatgctgccacttattactgccagcagtggagtagtaacccacagtggacgttcggtggaggcaccaagctggaaatcaaa

SEQ ID NO: 81 - protein, 10 aa, Artificial Sequence
GFSLTTSGMG

SEQ ID NO: 82 - DNA, 30 bp, Artificial Sequence
  source 1..30: mol_type = other DNA
gggttttcactgaccacttctggtatgggt

SEQ ID NO: 83 - protein, 7 aa, Artificial Sequence
MWWDDDK

SEQ ID NO: 84 - DNA, 21 bp, Artificial Sequence
  source 1..21: mol_type = other DNA
atgtggtgggatgacgataag

SEQ ID NO: 85 - protein, 11 aa, Artificial Sequence
ARRVYSSWFAY

SEQ ID NO: 86 - DNA, 33 bp, Artificial Sequence
  source 1..33: mol_type = other DNA
gctcgaagagtctacagtagttggtttgcttac

SEQ ID NO: 87 - protein, 6 aa, Artificial Sequence
QNVGAN

SEQ ID NO: 88 - DNA, 18 bp, Artificial Sequence
  source 1..18: mol_type = other DNA
cagaatgtgggtgctaat

SEQ ID NO: 89-90 - skipped (2 entries)

SEQ ID NO: 91 - protein, 9 aa, Artificial Sequence
QQYNNYPLT

SEQ ID NO: 92 - DNA, 27 bp, Artificial Sequence
  source 1..27: mol_type = other DNA
cagcaatataacaactatcctctcacg

SEQ ID NO: 93 - protein, 119 aa, Artificial Sequence
QVTLKESGPGILQPSQTLSLTCSFSGFSLTTSGMGVGWIRQPSGKGLEWLADMWWDDDKNYNPSLKSRLTISKDNSKKQVFLKIASVDTADTATYYCARRVYSSWFAYWGQGTLVTVSA

SEQ ID NO: 94 - DNA, 357 bp, Artificial Sequence
  source 1..357: mol_type = other DNA
caggttactctgaaagagtctggccctggaatattgcagccctcccagaccctcagtctgacttgttctttctctgggttttcactgaccacttctggtatgggtgtaggctggattcgtcagccttcaggaaagggtctagagtggctggcagacatgtggtgggatgacgataagaattataatccatccctgaagagccggctcacaatctccaaggataactccaaaaagcaggtattcctcaagatcgccagtgtggacactgcagatactgccacttactactgtgctcgaagagtctacagtagttggtttgcttactggggccaagggactctggtcactgtctctgca

SEQ ID NO: 95 - protein, 109 aa, Artificial Sequence
DGDIVMTQSQKFMSTSVGDRVSVTCKASQNVGANVAWYQQKPGQSPKTLIYSASYRYGGVPDRFTGSGSGTDFTFTITNVQSEDLAEYFCQQYNNYPLTFGAGTKLDLK

SEQ ID NO: 96 - DNA, 327 bp, Artificial Sequence
  source 1..327: mol_type = other DNA
gatggagacattgtgatgacccagtctcaaaaattcatgtccacatcagtaggagacagggtcagcgtcacctgcaaggccagtcagaatgtgggtgctaatgtagcctggtatcaacagaaaccagggcaatctcctaaaacactgatttattcggcatcctaccggtacggtggagtccctgatcgcttcacaggcagtggatctgggacagatttcactttcaccatcactaatgtgcagtctgaagacttggcagagtatttctgtcagcaatataacaactatcctctcacgttcggtgctgggaccaagttggacctgaaa

SEQ ID NO: 97 - protein, 8 aa, Artificial Sequence
GYTLSSYW

SEQ ID NO: 98 - DNA, 24 bp, Artificial Sequence
  source 1..24: mol_type = other DNA
ggctacactttaagtagttattgg

SEQ ID NO: 99 - protein, 8 aa, Artificial Sequence
INPSNNYT

SEQ ID NO: 100 - DNA, 24 bp, Artificial Sequence
  source 1..24: mol_type = other DNA
attaatcctagcaataattatact

SEQ ID NO: 101 - protein, 5 aa, Artificial Sequence
ATWGY

SEQ ID NO: 102 - DNA, 15 bp, Artificial Sequence
  source 1..15: mol_type = other DNA
gcaacatggggctac

SEQ ID NO: 103 - protein, 6 aa, Artificial Sequence
QDVSTA

SEQ ID NO: 104 - DNA, 18 bp, Artificial Sequence
  source 1..18: mol_type = other DNA
caggatgtgagtactgct

SEQ ID NO: 105-106 - skipped (2 entries)

SEQ ID NO: 107 - protein, 9 aa, Artificial Sequence
QHHYTTTWT

SEQ ID NO: 108 - DNA, 27 bp, Artificial Sequence
  source 1..27: mol_type = other DNA
cagcaccattatactactacgtggacg

SEQ ID NO: 109 - protein, 112 aa, Artificial Sequence
QVQLQQSGAELTKPGTSVKMSCKASGYTLSSYWMNWIKQRPGQGLEWIGTINPSNNYTAYNLKFKDKAMLTADKSSSTAYMQLSSLTSEDSAVYYCATWGYWGQGTTLTVSS

SEQ ID NO: 110 - DNA, 336 bp, Artificial Sequence
  source 1..336: mol_type = other DNA
caggtccagctgcagcagtctggcgctgaactgacaaaacctgggacctcagtgaagatgtcctgcaaggcctctggctacactttaagtagttattggatgaactggataaaacagaggcctggacaaggtctggaatggattgggactattaatcctagcaataattatactgcatacaatctgaagtttaaggacaaggccatgttgactgcagacaaatcctccagtacagcctacatgcaactcagcagcctgacatctgaggactctgcagtctattactgtgcaacatggggctactggggccaaggcaccactctcacagtctcctca

SEQ ID NO: 111 - protein, 107 aa, Artificial Sequence
DIVMTQSHKFMSTSVGDRVSITCKASQDVSTAVAWHQQKPGQPPKLLIYSASYRYTGVPDRFTGSGSGTDFTFTISSVQTEDLAIYYCQHHYTTTWTFGGGTKLEIR

SEQ ID NO: 112 - DNA, 321 bp, Artificial Sequence
  source 1..321: mol_type = other DNA
gacattgtgatgacccagtctcacaaattcatgtccacatcagtaggagacagggtcagcatcacctgcaaggccagtcaggatgtgagtactgctgtagcctggcatcaacagaaaccaggacagcctcctaagctactgatttactcggcatcttaccggtacactggagtccctgatcgcttcactggcagtggatctgggacggatttcactttcaccatcagcagtgtgcagactgaagacctggcaatttattactgtcagcaccattatactactacgtggacgttcggtggaggcaccaagctggaaatcaga

SEQ ID NO: 113 - protein, 10 aa, Artificial Sequence
GFSLSTSVMG

SEQ ID NO: 114 - DNA, 30 bp, Artificial Sequence
  source 1..30: mol_type = other DNA
ggcttctctctgtccacatctgtgatgggc

SEQ ID NO: 115 - protein, 7 aa, Artificial Sequence
IWWDDDK

SEQ ID NO: 116 - DNA, 21 bp, Artificial Sequence
  source 1..21: mol_type = other DNA
atctggtgggacgacgataag

SEQ ID NO: 117 - protein, 15 aa, Artificial Sequence
ARAYYSNYEYYGMDY

SEQ ID NO: 118 - DNA, 45 bp, Artificial Sequence
  source 1..45: mol_type = other DNA
gcccgcgcttattactctaactacgagtactatggcatggattac

SEQ ID NO: 119 - protein, 11 aa, Artificial Sequence
QSIVHSNGNTY

SEQ ID NO: 120 - DNA, 33 bp, Artificial Sequence
  source 1..33: mol_type = other DNA
cagagcattgttcatagtaatggaaacacctat

SEQ ID NO: 121-122 - skipped (2 entries)

SEQ ID NO: 123 - protein, 9 aa, Artificial Sequence
FQGSHVPFT

SEQ ID NO: 124 - DNA, 27 bp, Artificial Sequence
  source 1..27: mol_type = other DNA
tttcaaggttcacatgttccattcacg

SEQ ID NO: 125 - protein, 123 aa, Artificial Sequence
QVTLKESGPGILQPSQTLSLTCSFSGFSLSTSVMGVGWIRQPSGKGLEWLADIWWDDDKDYNPSLKSRLTISKDTSKNQVFLKIASVDTADTATYYCARAYYSNYEYYGMDYWGQGTSVTVSS

SEQ ID NO: 126 - DNA, 369 bp, Artificial Sequence
  source 1..369: mol_type = other DNA
caggtcacactgaaagagtctggtcccggcatcctgcagccttctcagaccctgtctctgacctgtagcttctccggcttctctctgtccacatctgtgatgggcgtgggctggatcagacagccttctggcaagggcctggagtggctggctgacatctggtgggacgacgataaggattacaacccttccctgaagtctcggctgaccatcagcaaggatacatccaagaatcaggtgttcctgaagatcgcttctgtggacaccgccgacaccgccacatattactgtgcccgcgcttattactctaactacgagtactatggcatggattactggggccagggcacatctgtgacagtgtcttcc

SEQ ID NO: 127 - protein, 112 aa, Artificial Sequence
DVLMTQTPLSLPVSLGDQASISCRSSQSIVHSNGNTYLEWYLQKPGQSPKLLIYKVSNRFSGVPDRFSGSGSGTDFTLKISRVEAEDLGVYYCFQGSHVPFTFGSGTKLEIK

SEQ ID NO: 128 - DNA, 336 bp, Artificial Sequence
  source 1..336: mol_type = other DNA
gatgttttgatgacccaaactccactctccctgcctgtcagtcttggagatcaagcctccatctcttgcagatctagtcagagcattgttcatagtaatggaaacacctatttagaatggtacctgcagaaaccaggccagtctccaaagctcctgatctacaaggtttccaaccgattttctggggtcccagacaggttcagtggcagtggatcagggacagatttcacactcaagatcagcagagtggaggctgaggatctgggagtttattactgctttcaaggttcacatgttccattcacgttcggctcggggacaaagttggaaataaaa

SEQ ID NO: 129 - protein, 10 aa, Artificial Sequence
GFSLSTSVMG

SEQ ID NO: 130 - DNA, 24 bp, Artificial Sequence
  source 1..24: mol_type = other DNA
gggttttcactgagtacttctgtt

SEQ ID NO: 131 - protein, 7 aa, Artificial Sequence
IWWDDDK

SEQ ID NO: 132 - DNA, 21 bp, Artificial Sequence
  source 1..21: mol_type = other DNA
atttggtgggatgacgataag

SEQ ID NO: 133 - protein, 15 aa, Artificial Sequence
ARTYYSNYEYYGMDY

SEQ ID NO: 134 - DNA, 45 bp, Artificial Sequence
  source 1..45: mol_type = other DNA
gctcgaacctactatagtaactacgaatactatggtatggactac

SEQ ID NO: 135 - protein, 11 aa, Artificial Sequence
QTIILSNGNTY

SEQ ID NO: 136 - DNA, 33 bp, Artificial Sequence
  source 1..33: mol_type = other DNA
cagaccattatacttagtaatggaaacacctat

SEQ ID NO: 137-138 - skipped (2 entries)

SEQ ID NO: 139 - protein, 9 aa, Artificial Sequence
FQGSHVPFT

SEQ ID NO: 140 - DNA, 27 bp, Artificial Sequence
  source 1..27: mol_type = other DNA
tttcaaggttcacatgttccattcacg

SEQ ID NO: 141 - protein, 123 aa, Artificial Sequence
QVTLKESGPGILQPSQTLSLTCSFSGFSLSTSVMGVGWIRQPSGKGLEWLADIWWDDDKDYNPSLKSRLTISKDTSKNQVFLKIASVDTADTATYYCARTYYSNYEYYGMDYWGQGTSVTVSS

SEQ ID NO: 142 - DNA, 369 bp, Artificial Sequence
  source 1..369: mol_type = other DNA
caggttactctgaaagagtctggccctggaatattgcagccctcccagaccctcagtctgacttgttctttctctgggttttcactgagtacttctgttatgggtgtaggctggattcgtcagccttcaggaaagggtctagagtggctggcagacatttggtgggatgacgataaggactataacccatccctgaagagccggctcacaatctccaaggatacctccaaaaaccaggtattcctcaagatcgccagtgtggacactgcagatactgccacttactactgtgctcgaacctactatagtaactacgaatactatggtatggactactggggtcaaggaacctcagtcaccgtctcctca

SEQ ID NO: 143 - protein, 112 aa, Artificial Sequence
DVLMTQTPLSLPVSLGDQASISCRSSQTIILSNGNTYLEWYLQKPGQSPKLLIYKVSNRFSGVPDRFSGSGSGTDFTLKISRVEAEDLGVYYCFQGSHVPFTFGSGTKLEIK

SEQ ID NO: 144 - DNA, 336 bp, Artificial Sequence
  source 1..336: mol_type = other DNA
gacgttttgatgacccaaactccactctccctgcctgtcagtcttggagatcaagcctccatctcttgcagatctagtcagaccattatacttagtaatggaaacacctatttagaatggtacctgcagaaaccaggccagtctccaaagctcctgatctacaaagtttccaaccgattttctggggtcccagacaggttcagtggcagtggatcggggacagatttcacactcaagatcagcagagtggaggctgaggatctgggagtttattactgttttcaaggttcacatgttccattcacgttcggctcggggacaaagttagaaataaaa

SEQ ID NO: 145 - protein, 8 aa, Artificial Sequence
GYTFTDYY

SEQ ID NO: 146 - DNA, 24 bp, Artificial Sequence
  source 1..24: mol_type = other DNA
ggatacacattcactgactactac

SEQ ID NO: 147 - protein, 8 aa, Artificial Sequence
INPINGDI

SEQ ID NO: 148 - DNA, 24 bp, Artificial Sequence
  source 1..24: mol_type = other DNA
attaatccgatcaatggtgatatt

SEQ ID NO: 149 - protein, 15 aa, Artificial Sequence
AREAFFGYKGNYFDY

SEQ ID NO: 150 - DNA, 45 bp, Artificial Sequence
  source 1..45: mol_type = other DNA
gcaagagaggctttctttggttacaaggggaactactttgactac

SEQ ID NO: 151 - protein, 10 aa, Artificial Sequence
ESVDNYGISF

SEQ ID NO: 152 - DNA, 30 bp, Artificial Sequence
  source 1..30: mol_type = other DNA
gaaagtgttgataattatggcattagtttt

SEQ ID NO: 153-154 - skipped (2 entries)

SEQ ID NO: 155 - protein, 9 aa, Artificial Sequence
QQTKEVPYT

SEQ ID NO: 156 - DNA, 27 bp, Artificial Sequence
  source 1..27: mol_type = other DNA
cagcaaactaaggaggttccgtacacg

SEQ ID NO: 157 - protein, 122 aa, Artificial Sequence
EVQLQQSGPELVMPGSSVKISCKASGYTFTDYYMNWVRQSHGKSLEWIGDINPINGDITYNQKFKGKATLTVDKSSSTDYMELRGLTSEDSAVYYCAREAFFGYKGNYFDYWGQGTTLTVSS

SEQ ID NO: 158 - DNA, 366 bp, Artificial Sequence
  source 1..366: mol_type = other DNA
gaggtccagctgcaacagtctgggcctgagctggtgatgcctgggtcttcagtgaagatatcatgtaaggcttctggatacacattcactgactactacatgaactgggtgaggcagagccatggaaagagccttgagtggattggagatattaatccgatcaatggtgatattacctacaaccagaagttcaagggcaaggccacattgactgtagacaagtcctccagcacagactacatggagctccgcggcctgacatctgaggactctgcagtctattactgtgcaagagaggctttctttggttacaaggggaactactttgactactggggccaaggcaccactctcacagtctcctca

SEQ ID NO: 159 - protein, 111 aa, Artificial Sequence
DIVLTQSPASLAVSLGQRATISCRASESVDNYGISFMSWFQQKPGQPPKLLIYAASNQGSGVPAKFSGSGSGTDFSLNIHPMEEDDPAMYFCQQTKEVPYTFGGGTKLEIK

SEQ ID NO: 160 - DNA, 333 bp, Artificial Sequence
  source 1..333: mol_type = other DNA
gacattgtgctgacccaatctccagcttctttggctgtgtctctagggcagagggccaccatctcctgcagagccagcgaaagtgttgataattatggcattagttttatgagctggttccaacagaaaccaggacagccacccaaactcctcatctatgctgcatccaaccaaggatccggggtccctgccaagtttagtggcagtgggtctgggacagacttcagcctcaacatccatcctatggaggaggatgatcctgcaatgtatttctgtcagcaaactaaggaggttccgtacacgttcggaggggggaccaagctggaaataaaa

SEQ ID NO: 161 - protein, 10 aa, Artificial Sequence
GFSLSTSVMG

SEQ ID NO: 162 - DNA, 30 bp, Artificial Sequence
  source 1..30: mol_type = other DNA
gggttttcactgagtacttctgttatgggt

SEQ ID NO: 163 - protein, 7 aa, Artificial Sequence
IWWDDDK

SEQ ID NO: 164 - DNA, 21 bp, Artificial Sequence
  source 1..21: mol_type = other DNA
atttggtgggatgacgataag

SEQ ID NO: 165 - protein, 15 aa, Artificial Sequence
ARAYYSNFEYYGMDY

SEQ ID NO: 166 - DNA, 45 bp, Artificial Sequence
  source 1..45: mol_type = other DNA
gctcgagcctactatagtaacttcgaatactatggtatggactac

SEQ ID NO: 167 - protein, 11 aa, Artificial Sequence
QTIVHSNGNTY

SEQ ID NO: 168 - DNA, 33 bp, Artificial Sequence
  source 1..33: mol_type = other DNA
cagaccattgtacatagtaatggaaacacctat

SEQ ID NO: 169-170 - skipped (2 entries)

SEQ ID NO: 171 - protein, 9 aa, Artificial Sequence
FQGSHVPFT

SEQ ID NO: 172 - DNA, 27 bp, Artificial Sequence
  source 1..27: mol_type = other DNA
tttcaaggttcacatgttccattcacg

SEQ ID NO: 173 - protein, 123 aa, Artificial Sequence
QVTLKESGPGILQPSQTLSLTCSFSGFSLSTSVMGVGWIRQPSGKGLEWLADIWWDDDKDYNPSLKSRLTISKDTSKNQVFLKIASVDTADTATYYCARAYYSNFEYYGMDYWGQGTSVTVSS

SEQ ID NO: 174 - DNA, 369 bp, Artificial Sequence
  source 1..369: mol_type = other DNA
caggttactctgaaagagtctggccctggaatattgcagccctcccagaccctcagtctgacttgttctttctctgggttttcactgagtacttctgttatgggtgtaggctggattcgtcagccttcaggaaagggtcttgagtggctggcagacatttggtgggatgacgataaggactataacccatctctgaagagccggctcacaatctccaaggatacctccaaaaaccaggtattcctcaagatcgccagtgtggacactgcagatactgccacttactactgtgctcgagcctactatagtaacttcgaatactatggtatggactactggggtcaaggaacctcagtcaccgtctcctca

SEQ ID NO: 175 - protein, 112 aa, Artificial Sequence
DVLMTQIPLSLPVSLGDQASISCRSSQTIVHSNGNTYLEWYLQKPGQSPKLLIYKVSNRFSGVPDRFSGSGSGTDFTLKISRVEAEDLGVYYCFQGSHVPFTFGSGTKLEIK

SEQ ID NO: 176 - DNA, 336 bp, Artificial Sequence
  source 1..336: mol_type = other DNA
gatgttttgatgacccaaattccactctccctgcctgtcagtcttggagatcaagcctccatctcttgcagatctagtcagaccattgtacatagtaatggaaacacctatttagaatggtacctgcagaaaccaggccagtctccaaagctcctgatctacaaagtttccaaccgattttctggggtcccagacaggttcagtggcagtggatcggggacagatttcacactcaagatcagcagagtggaggctgaggatctgggagtttattactgctttcaaggttcacatgttccattcacgttcggctcggggacaaagttggaaataaaa

SEQ ID NO: 177 - protein, 10 aa, Artificial Sequence
GYTFTTYWMN

SEQ ID NO: 178 - DNA, 30 bp, Artificial Sequence
  source 1..30: mol_type = other DNA
ggctacacctttactacctactggatgaac

SEQ ID NO: 179 - protein, 8 aa, Artificial Sequence
INPSNDYT

SEQ ID NO: 180 - DNA, 24 bp, Artificial Sequence
  source 1..24: mol_type = other DNA
attaatcctagcaatgattatact

SEQ ID NO: 181 - protein, 8 aa, Artificial Sequence
GRSYSPDY

SEQ ID NO: 182 - DNA, 24 bp, Artificial Sequence
  source 1..24: mol_type = other DNA
ggaaggagttactcccctgactac

SEQ ID NO: 183 - protein, 6 aa, Artificial Sequence
QNVDNH

SEQ ID NO: 184 - DNA, 18 bp, Artificial Sequence
  source 1..18: mol_type = other DNA
cagaatgtggataatcat

SEQ ID NO: 185-186 - skipped (2 entries)

SEQ ID NO: 187 - protein, 9 aa, Artificial Sequence
QQYKSYPFT

SEQ ID NO: 188 - DNA, 27 bp, Artificial Sequence
  source 1..27: mol_type = other DNA
cagcaatataaaagctatccattcacg

SEQ ID NO: 189 - protein, 115 aa, Artificial Sequence
QVQLQQSGAELAKPGTSVKMSCKASGYTFTTYWMNWVKQRPGQDLEWIGAINPSNDYTEYNQKFKDKAILTADKSSNTAYMQLSSLTSEDSAVYYCGRSYSPDYWGQGTTLTVSS

SEQ ID NO: 190 - DNA, 345 bp, Artificial Sequence
  source 1..345: mol_type = other DNA
caggtccagctgcagcagtctggcgctgaactggcaaaacctgggacctcagtgaagatgtcctgcaaggcttctggctacacctttactacctactggatgaactgggtaaaacagaggcctggacaggatctggaatggattggggctattaatcctagcaatgattatactgagtacaatcagaagttcaaggacaaggccatattgactgcagacaaatcctccaacacagcctacatgcaactgagtagcctgacatctgaggactctgcagtctattactgtggaaggagttactcccctgactactggggccaaggcaccactctcacagtctcatca

SEQ ID NO: 191 - protein, 107 aa, Artificial Sequence
DIVMTQSQKFMSTSVGDRVSVTCKASQNVDNHVAWHQQKPGQSPKALIYSASYRYSGVPDRFTGSGSGTDFTLTIRDVQSEDLADYFCQQYKSYPFTFGSGTELEIK

SEQ ID NO: 192 - DNA, 321 bp, Artificial Sequence
  source 1..321: mol_type = other DNA
gacattgtgatgacccagtctcaaaaattcatgtccacatcagtaggagacagggtcagcgtcacctgcaaggccagtcagaatgtggataatcatgtagcctggcatcaacagaaaccagggcagtctcctaaggcactgatttactcggcatcctaccggtacagtggagtccctgatcgcttcacaggcagtggatctgggacagatttcactctcaccatccgcgatgtgcagtctgaagacttggcagactatttctgtcagcaatataaaagctatccattcacgttcggctcggggacagagttggaaataaaa

SEQ ID NO: 193 - protein, 8 aa, Artificial Sequence
GFNIKDYY

SEQ ID NO: 194 - DNA, 24 bp, Artificial Sequence
  source 1..24: mol_type = other DNA
ggcttcaacattaaagactactat

SEQ ID NO: 195 - protein, 8 aa, Artificial Sequence
IDPENGDT

SEQ ID NO: 196 - DNA, 24 bp, Artificial Sequence
  source 1..24: mol_type = other DNA
attgatcctgagaatggtgatact

SEQ ID NO: 197 - protein, 13 aa, Artificial Sequence
NGVYYGSRGFFDY

SEQ ID NO: 198 - DNA, 39 bp, Artificial Sequence
  source 1..39: mol_type = other DNA
aatggagtttactacggtagtagagggttctttgactac

SEQ ID NO: 199 - protein, 11 aa, Artificial Sequence
QSLLDSDGKTY

SEQ ID NO: 200 - DNA, 33 bp, Artificial Sequence
  source 1..33: mol_type = other DNA
cagagcctcttagatagtgatggaaagacatat

SEQ ID NO: 201-202 - skipped (2 entries)

SEQ ID NO: 203 - protein, 9 aa, Artificial Sequence
CQITHFPFT

SEQ ID NO: 204 - DNA, 27 bp, Artificial Sequence
  source 1..27: mol_type = other DNA
tgccaaattacacattttccattcacg

SEQ ID NO: 205 - protein, 120 aa, Artificial Sequence
EVQLQQSGAELVRSGASVKLSCTASGFNIKDYYMHWVKQRPDQGLEWIGWIDPENGDTEYAPKFQGKATMTADTSPNTAYLQLSSLTSEDTAVYYCNGVYYGSRGFFDYWGQGTTLTVSS

SEQ ID NO: 206 - DNA, 360 bp, Artificial Sequence
  source 1..360: mol_type = other DNA
gaggttcagctgcagcagtctggggcagagcttgtgaggtcaggggcctcagtcaagttgtcctgcacagcttctggcttcaacattaaagactactatatgcactgggtgaagcagaggcctgatcagggcctggagtggattggatggattgatcctgagaatggtgatactgaatacgccccgaagttccagggcaaggccactatgactgcagacacatcccccaacacagcctacctgcagctcagcagcctgacatctgaggacactgccgtctattactgtaatggagtttactacggtagtagagggttctttgactactggggccaaggcaccactctcacagtctcctca

SEQ ID NO: 207 - protein, 112 aa, Artificial Sequence
DVVMTQTPLTLSVTIGQPASISCKSSQSLLDSDGKTYLNWLLQRPGQSPKRLIYLVSKLDSGVPDRFTGSGSGTDFTLKISRVEAEDLGVYYCCQITHFPFTFGSGTKLEIK

SEQ ID NO: 208 - DNA, 336 bp, Artificial Sequence
  source 1..336: mol_type = other DNA
gatgttgtgatgacccagactccactcactttgtcggttaccattggacaaccagcctccatctcttgcaagtcaagtcagagcctcttagatagtgatggaaagacatatttgaattggttgttacagaggccaggccagtctccaaagcgcctaatctatctggtgtctaaactggactctggagtccctgacaggttcactggcagtggatcagggacagatttcacactgaaaatcagcagagtggaggctgaggatttgggagtttattattgctgccaaattacacattttccattcacgttcggctcggggacaaagttggaaataaaa

SEQ ID NO: 209 - protein, 572 aa, Homo sapiens
MECLYYFLGFLLLAARLPLDAAKRFHDVLGNERPSAYMREHNQLNGWSSDENDWNEKLYPVWKRGDMRWKNSWKGGRVQAVLTSDSPALVGSNITFAVNLIFPRCQKEDANGNIVYEKNCRNEAGLSADPYVYNWTAWSEDSDGENGTGQSHHNVFPDGKPFPHHPGWRRWNFIYVFHTLGQYFQKLGRCSVRVSVNTANVTLGPQLMEVTVYRRHGRAYVPIAQVKDVYVVTDQIPVFVTMFQKNDRNSSDETFLKDLPIMFDVLIHDPSHFLNYSTINYKWSFGDNTGLFVSTNHTVNHTYVLNGTFSLNLTVKAAAPGPCPPPPPPPRPSKPTPSLATTLKSYDSNTPGPAGDNPLELSRIPDENCQINRYGHFQATITIVEGILEVNIIQMTDVLMPVPWPESSLIDFVVTCQGSIPTEVCTIISDPTCEITQNTVCSPVDVDEMCLLTVRRTFNGSGTYCVNLTLGDDTSLALTSTLISVPDRDPASPLRMANSALISVGCLAIFVTVISLLVYKKHKEYNPIENSPGNVVRSKGLSVFLNRAKAVFFPGNQEKDPLLKNQEFKGVS

SEQ ID NO: 210 - DNA, 1719 bp, Homo sapiens
  source 1..1719: mol_type = other DNA
atggaatgtctctactatttcctgggatttctgctcctggctgcaagattgccacttgatgccgccaaacgatttcatgatgtgctgggcaatgaaagaccttctgcttacatgagggagcacaatcaattaaatggctggtcttctgatgaaaatgactggaatgaaaaactctacccagtgtggaagcggggagacatgaggtggaaaaactcctggaagggaggccgtgtgcaggcggtcctgaccagtgactcaccagccctcgtgggctcaaatataacatttgcggtgaacctgatattccctagatgccaaaaggaagatgccaatggcaacatagtctatgagaagaactgcagaaatgaggctggtttatctgctgatccgtatgtttacaactggacagcatggtcagaggacagtgacggggaaaatggcaccggccaaagccatcataacgtcttccctgatgggaaaccttttcctcaccaccccggatggagaagatggaatttcatctacgtcttccacacacttggtcagtatttccagaaattgggacgatgttcagtgagagtttctgtgaacacagccaatgtgacacttgggcctcaactcatggaagtgactgtctacagaagacatggacgggcatatgttcccatcgcacaagtgaaagatgtgtacgtggtaacagatcagattcctgtgtttgtgactatgttccagaagaacgatcgaaattcatccgacgaaaccttcctcaaagatctccccattatgtttgatgtcctgattcatgatcctagccacttcctcaattattctaccattaactacaagtggagcttcggggataatactggcctgtttgtttccaccaatcatactgtgaatcacacgtatgtgctcaatggaaccttcagccttaacctcactgtgaaagctgcagcaccaggaccttgtccgccaccgccaccaccacccagaccttcaaaacccaccccttctttagcaactactctaaaatcttatgattcaaacaccccaggacctgctggtgacaaccccctggagctgagtaggattcctgatgaaaactgccagattaacagatatggccactttcaagccaccatcacaattgtagagggaatcttagaggttaacatcatccagatgacagacgtcctgatgccggtgccatggcctgaaagctccctaatagactttgtcgtgacctgccaagggagcattcccacggaggtctgtaccatcatttctgaccccacctgcgagatcacccagaacacagtctgcagccctgtggatgtggatgagatgtgtctgctgactgtgagacgaaccttcaatgggtctgggacgtactgtgtgaacctcaccctgggggatgacacaagcctggctctcacgagcaccctgatttctgttcctgacagagacccagcctcgcctttaaggatggcaaacagcgccctgatctccgttggctgcttggccatatttgtcactgtgatctccctcttggtgtacaaaaaacacaaggaatacaacccaatagaaaatagtcctgggaatgtggtcagaagcaaaggcctgagtgtctttctcaaccgtgcaaaagccgtgttcttcccgggaaaccaggaaaaggatccgctactcaaaaaccaagaatttaaaggagtttcttaa

SEQ ID NO: 211 - protein, 574 aa, Mus musculus
MESLCGVLGFLLLAAGLPLQAAKRFRDVLGHEQYPNHMREHNQLRGWSSDENEWDEHLYPVWRRGDGRWKDSWEGGRVQAVLTSDSPALVGSNITFVVNLVFPRCQKEDANGNIVYEKNCRNDLGLTSDLHVYNWTAGADDGDWEDGTSRSQHLRFPDRRPFPRPHGWKKWSFVYVFHTLGQYFQKLGRCSARVSINTVNLTAGPQVMEVTVFRRYGRAYIPISKVKDVYVITDQIPVFVTMSQKNDRNLSDEIFLRDLPIVFDVLIHDPSHFLNDSAISYKWNFGDNTGLFVSNNHTLNHTYVLNGTFNLNLTVQTAVPGPCPPPSPSTPPPPSTPPSPPPSPLPTLSTPSPSLMPTGYKSMELSDISNENCRINRYGYFRATITIVEGILEVSIMQIADVPMPTPQPANSLMDFTVTCKGATPMEACTIISDPTCQIAQNRVCSPVAVDGLCLLSVRRAFNGSGTYCVNFTLGDDASLALTSTLISIPGKDPDSPLRAVNGVLISIGCLAVLVTMVTILLYKKHKAYKPIGNCPRNTVKGKGLSVLLSHAKAPFFRGDQEKDPLLQDKPRTL

SEQ ID NO: 212 - DNA, 1725 bp, Mus musculus
  source 1..1725: mol_type = other DNA
atggaaagtctctgcggggtcctgggatttctgctgctggctgcaggactgcctctccaggctgccaagcgatttcgtgatgtgctgggccatgaacagtatcccaatcacatgagagagcacaaccaattacgtggctggtcttcggatgaaaatgaatgggatgaacacctgtatccagtgtggaggaggggagacggcaggtggaaggactcctgggaaggaggccgtgtgcaggcagtcctgaccagtgactcaccggctctggtgggttccaatatcacctttgtggtgaacctggtgttccccagatgccagaaggaagatgctaatggcaatatcgtctatgagaagaactgcaggaatgatttgggactgacctctgacctgcatgtctacaactggactgcaggggcagatgatggtgactgggaagatggcaccagccgaagccagcatctcaggttcccggacaggaggcccttccctcgcccccatggatggaagaaatggagctttgtctacgtctttcacacacttggccagtatttccaaaaactgggtcggtgttcagcacgggtttctataaacacagtcaacttgacagctggccctcaggtcatggaagtgactgtctttcgaagatacggccgggcatacattcccatctcgaaggtgaaagatgtgtatgtgataacagatcagatccctgtattcgtgaccatgtcccagaagaatgacaggaacttgtctgatgagatcttcctcagagacctccccatcgtcttcgatgtcctcattcatgatcccagccacttcctcaacgactctgccatttcctacaagtggaactttggggacaacactggcctgtttgtctccaacaatcacactttgaatcacacttatgtgctcaatggaaccttcaaccttaacctcaccgtgcaaactgcagtgcccgggccatgccctcccccttcgccttcgactccgcctccaccttcaactccgccctcacctccgccctcacctctgcccacattatcaacacctagcccctctttaatgcctactggttacaaatccatggagctgagtgacatttccaatgaaaactgccgaataaacagatatggctacttcagagccaccatcacaattgtagaggggatcctggaagtcagcatcatgcagatagcagatgtccccatgcccacaccgcagcctgccaactccctgatggacttcactgtgacctgcaaaggggccacccccatggaagcctgtacgatcatctccgaccccacctgccagatcgcccagaaccgggtctgcagccctgtggctgtggatgggctgtgcctgctgtctgtgagaagagccttcaatgggtctggcacctactgtgtgaatttcactctgggagatgatgcaagcctggccctcaccagcaccctgatctctatccctggcaaagacccagactcccctctgagagcagtgaatggtgtcctgatctccattggctgcctggctgtgcttgtcaccatggttaccatcttgctgtacaaaaaacacaaggcgtacaagccaataggaaactgccccaggaacacggtcaagggcaaaggcctgagtgttctcctcagccacgcgaaagccccgttcttccgaggagaccaggagaaggatccattgctccaggacaagccaaggacactctaa

SEQ ID NO: 213 - protein, 572 aa, Rattus norvegicus
MESLCGVLVFLLLAAGLPLQAAKRFRDVLGHEQYPDHMRENNQLRGWSSDENEWDEQLYPVWRRGEGRWKDSWEGGRVQAALTSDSPALVGSNITFVVNLVFPRCQKEDANGNIVYERNCRSDLELASDPYVYNWTTGADDEDWEDSTSQGQHLRFPDGKPFPRPHGRKKWNFVYVFHTLGQYFQKLGRCSARVSINTVNLTVGPQVMEVIVFRRHGRAYIPISKVKDVYVITDQIPIFVTMYQKNDRNSSDETFLRDLPIFFDVLIHDPSHFLNYSAISYKWNFGDNTGLFVSNNHTLNHTYVLNGTFNFNLTVQTAVPGPCPSPTPSPSSSTSPSPASSPSPTLSTPSPSLMPTGHKSMELSDISNENCRINRYGYFRATITIVDGILEVNIIQVADVPIPTPQPDNSLMDFIVTCKGATPTEACTIISDPTCQIAQNRVCSPVAVDELCLLSVRRAFNGSGTYCVNFTLGDDASLALTSALISIPGKDLGSPLRTVNGVLISIGCLAMFVTMVTILLYKKHKTYKPIGNCTRNVVKGKGLSVFLSHAKAPFSRGDREKDPLLQDKPWML

SEQ ID NO: 214 - DNA, 1719 bp, Rattus norvegicus
  source 1..1719: mol_type = other DNA
atggaaagtctctgcggggtcctggtatttctgctgctggctgcaggactgccgctccaggcggccaagcggttccgtgatgtgctgggccatgagcagtatccggatcacatgagggagaacaaccaattacgtggctggtcttcagatgaaaatgaatgggatgaacagctgtatccagtgtggaggaggggagagggcagatggaaggactcctgggaaggaggccgtgtgcaggcagccctaaccagtgattcaccggccttggtgggttccaatatcaccttcgtagtgaacctggtgttccccagatgccagaaggaagatgccaacggcaatatcgtctatgagaggaactgcagaagtgatttggagctggcttctgacccgtatgtctacaactggaccacaggggcagacgatgaggactgggaagacagcaccagccaaggccagcacctcaggttccccgacgggaagcccttccctcgcccccacggacggaagaaatggaacttcgtctacgtcttccacacacttggtcagtattttcaaaagctgggtcggtgttcagcacgagtttctataaacacagtcaacttgacagttggccctcaggtcatggaagtgattgtctttcgaagacacggccgggcatacattcccatctccaaagtgaaagacgtgtatgtgataacagatcagatccctatattcgtgaccatgtaccagaagaatgaccggaactcgtctgatgaaaccttcctcagagacctccccattttcttcgatgtcctcattcacgatcccagtcatttcctcaactactctgccatttcctacaagtggaactttggggacaacactggcctgtttgtctccaacaatcacactttgaatcacacgtatgtgctcaatggaaccttcaactttaacctcaccgtgcaaactgcagtgccgggaccatgcccctcacccacaccttcgccttcttcttcgacttctccttcgcctgcatcttcgccttcacccacattatcaacacctagtccctctttaatgcctactggccacaaatccatggagctgagtgacatttccaatgaaaactgccgaataaacagatatggttacttcagagccaccatcacaattgtagatggaatcctagaagtcaacatcatccaggtagcagatgtcccaatccccacaccgcagcctgacaactcactgatggacttcattgtgacctgcaaaggggccactcccacggaagcctgtacgatcatctctgaccccacctgccagatcgcccagaacagggtgtgcagcccggtggctgtggatgagctgtgcctcctgtccgtgaggagagccttcaatgggtccggcacgtactgtgtgaatttcactctgggagacgatgcaagcctggccctcaccagcgccctgatctctatccctggcaaagacctaggctcccctctgagaacagtgaatggtgtcctgatctccattggctgcctggccatgtttgtcaccatggttaccatcttgctgtacaaaaaacacaagacgtacaagccaataggaaactgcaccaggaacgtggtcaagggcaaaggcctgagtgtttttctcagccatgcaaaagccccgttctcccgaggagaccgggagaaggatccactgctccaggacaagccatggatgctctaa

SEQ ID NO: 215 - protein, 498 aa, Homo sapiens
MECLYYFLGFLLLAARLPLDAAKRFHDVLGNERPSAYMREHNQLNGWSSDENDWNEKLYPVWKRGDMRWKNSWKGGRVQAVLTSDSPALVGSNITFAVNLIFPRCQKEDANGNIVYEKNCRNEAGLSADPYVYNWTAWSEDSDGENGTGQSHHNVFPDGKPFPHHPGWRRWNFIYVFHTLGQYFQKLGRCSVRVSVNTANVTLGPQLMEVTVYRRHGRAYVPIAQVKDVYVVTDQIPVFVTMFQKNDRNSSDETFLKDLPIMFDVLIHDPSHFLNYSTINYKWSFGDNTGLFVSTNHTVNHTYVLNGTFSLNLTVKAAAPGPCPPPPPPPRPSKPTPSLATTLKSYDSNTPGPAGDNPLELSRIPDENCQINRYGHFQATITIVEGILEVNIIQMTDVLMPVPWPESSLIDFVVTCQGSIPTEVCTIISDPTCEITQNTVCSPVDVDEMCLLTVRRTFNGSGTYCVNLTLGDDTSLALTSTLISVPDRDPASPLRMAN

SEQ ID NO: 216 - DNA, 1494 bp, Homo sapiens
  source 1..1494: mol_type = other DNA
atggaatgtctctactatttcctgggatttctgctcctggctgcaagattgccacttgatgccgccaaacgatttcatgatgtgctgggcaatgaaagaccttctgcttacatgagggagcacaatcaattaaatggctggtcttctgatgaaaatgactggaatgaaaaactctacccagtgtggaagcggggagacatgaggtggaaaaactcctggaagggaggccgtgtgcaggcggtcctgaccagtgactcaccagccctcgtgggctcaaatataacatttgcggtgaacctgatattccctagatgccaaaaggaagatgccaatggcaacatagtctatgagaagaactgcagaaatgaggctggtttatctgctgatccgtatgtttacaactggacagcatggtcagaggacagtgacggggaaaatggcaccggccaaagccatcataacgtcttccctgatgggaaaccttttcctcaccaccccggatggagaagatggaatttcatctacgtcttccacacacttggtcagtatttccagaaattgggacgatgttcagtgagagtttctgtgaacacagccaatgtgacacttgggcctcaactcatggaagtgactgtctacagaagacatggacgggcatatgttcccatcgcacaagtgaaagatgtgtacgtggtaacagatcagattcctgtgtttgtgactatgttccagaagaacgatcgaaattcatccgacgaaaccttcctcaaagatctccccattatgtttgatgtcctgattcatgatcctagccacttcctcaattattctaccattaactacaagtggagcttcggggataatactggcctgtttgtttccaccaatcatactgtgaatcacacgtatgtgctcaatggaaccttcagccttaacctcactgtgaaagctgcagcaccaggaccttgtccgccaccgccaccaccacccagaccttcaaaacccaccccttctttagcaactactctaaaatcttatgattcaaacaccccaggacctgctggtgacaaccccctggagctgagtaggattcctgatgaaaactgccagattaacagatatggccactttcaagccaccatcacaattgtagagggaatcttagaggttaacatcatccagatgacagacgtcctgatgccggtgccatggcctgaaagctccctaatagactttgtcgtgacctgccaagggagcattcccacggaggtctgtaccatcatttctgaccccacctgcgagatcacccagaacacagtctgcagccctgtggatgtggatgagatgtgtctgctgactgtgagacgaaccttcaatgggtctgggacgtactgtgtgaacctcaccctgggggatgacacaagcctggctctcacgagcaccctgatttctgttcctgacagagacccagcctcgcctttaaggatggcaaac

SEQ ID NO: 217 - protein, 502 aa, Mus musculus
MESLCGVLGFLLLAAGLPLQAAKRFRDVLGHEQYPDHMREHNQLRGWSSDENEWDEHLYPVWRRGDGRWKDSWEGGRVQAVLTSDSPALVGSNITFVVNLVFPRCQKEDANGNIVYEKNCRNDLGLTSDLHVYNWTAGADDGDWEDGTSRSQHLRFPDRRPFPRPHGWKKWSFVYVFHTLGQYFQKLGRCSARVSINTVNLTAGPQVMEVTVFRRYGRAYIPISKVKDVYVITDQIPVFVTMSQKNDRNLSDEIFLRDLPIVFDVLIHDPSHFLNDSAISYKWNFGDNTGLFVSNNHTLNHTYVLNGTFNLNLTVQTAVPGPCPPPSPSTPPPPSTPPSPPPSPLPTLSTPSPSLMPTGYKSMELSDISNENCRINRYGYFRATITIVEGILEVSIMQIADVPMPTPQPANSLMDFTVTCKGATPMEACTIISDPTCQIAQNRVCSPVAVDGLCLLSVRRAFNGSGTYCVNFTLGDDASLALTSTLISIPGKDPDSPLRAVN

SEQ ID NO: 218 - DNA, 1506 bp, Mus musculus
  source 1..1506: mol_type = other DNA
atggaaagtctctgcggggtcctgggatttctgctgctggctgcaggactgcctctccaggctgccaagcgatttcgtgatgtgctgggccatgaacagtatcccgatcacatgagagagcacaaccaattacgtggctggtcttcggatgaaaatgaatgggatgaacacctgtatccagtgtggaggaggggagacggcaggtggaaggactcctgggaaggaggccgtgtgcaggcagtcctgaccagtgactcaccggctctggtgggttccaatatcacttttgtggtgaacctggtgttccccagatgccagaaggaagatgctaatggcaatatcgtctatgagaagaactgcaggaatgatttgggactgacatctgacctgcatgtctacaactggactgcaggggcagatgatggtgactgggaagatggcaccagccgaagccagcatctcaggttcccggacaggaggcccttccctcgcccccatggatggaagaaatggagctttgtctacgtctttcacacacttggccagtatttccaaaaactgggtcggtgttcagcacgggtttctataaacacagtcaacttgacagctggccctcaggtcatggaagtgactgtctttcgaagatacggccgggcatacattcccatctcgaaggtgaaagatgtgtatgtgataacagatcagatccctgtattcgtgaccatgtcccagaagaatgacaggaacttgtctgatgagatcttcctcagagacctccccatcgtcttcgatgtcctcattcatgatcccagccacttcctcaacgactctgccatttcctacaagtggaactttggggacaacactggcctgtttgtctccaacaatcacactttgaatcacacttatgtgctcaatggaaccttcaaccttaacctcaccgtgcaaactgcagtgcccgggccatgccctcccccttcgccttcgactccgcctccaccttcaactccgccctcacctccgccctcacctctgcccacattatcaacacctagcccctctttaatgcctactggttacaaatccatggagctgagtgacatttccaatgaaaactgccgaataaacagatatggctacttcagagccaccatcacaattgtagaggggatcctggaagtcagcatcatgcagatagcagatgtccccatgcccacaccgcagcctgccaactccctgatggacttcactgtgacctgcaaaggggccacccccatggaagcctgtacgatcatctccgaccccacctgccagatcgcccagaaccgggtctgcagccctgtggctgtggatgggctgtgcctgctgtctgtgagaagagccttcaatgggtctggcacctactgtgtgaatttcactctgggagatgatgcaagcctggccctcaccagcaccctgatctctatccctggcaaagacccagactcccctctgagagcagtgaat

SEQ ID NO: 219 - protein, 500 aa, Rattus norvegicus
MESLCGVLVFLLLAAGLPLQAAKRFRDVLGHEQYPDHMRENNQLRGWSSDENEWDEQLYPVWRRGEGRWKDSWEGGRVQAALTSDSPALVGSNITFVVNLVFPRCQKEDANGNIVYERNCRSDLELASDPYVYNWTTGADDEDWEDNTSQGQHLRFPDGKPFPRPHGRKKWNFVYVFHTLGQYFQKLGQCSARVSINTVNLTVGPQVMEVIVFRRHGRAYIPISKVKDVYVITDQIPIFVTMYQKNDRNSSDETFLRDLPIFFDVLIHDPSHFLNYSAISYKWNFGDNTGLFVSNNHTLNHTYVLNGTFNFNLTVQTAVPGPCPSPTPSPSSSTSPSPASSPSPTLSTPSPSLMPTGYKSMELSDISNENCRINRYGYFRATITIVDGILEVNIIQVADVPIPTLQPDNSLMDFIVTCKGATPTEACTIISDPTCQIAQNRVCSPVAVDELCLLSVRRAFNGSGTYCVNFTLGDDASLALTSALISIPGKDLGSPLRTVN

SEQ ID NO: 220 - DNA, 1500 bp, Rattus norvegicus
  source 1..1500: mol_type = other DNA
atggaaagtctctgcggggtcctggtatttctgctgctggctgcaggactgccgctccaggcggccaagcggttccgtgatgtgctgggccatgagcagtatccggatcacatgagggagaacaaccaattacgtggctggtcttcagatgaaaatgaatgggatgaacagctgtatccagtgtggaggaggggagagggcagatggaaggactcctgggaaggaggccgtgtgcaggcagccctaaccagtgattcaccggccttggtgggttccaatatcaccttcgtagtgaacctggtgttccccagatgccagaaggaagatgccaacggcaatatcgtctatgagaggaactgcagaagtgatttggagctggcttctgacccgtatgtctacaactggaccacaggggcagacgatgaggactgggaagacaacaccagccaaggccagcacctcaggttccccgacgggaagcccttccctcgcccccacggacggaagaaatggaacttcgtctacgtcttccacacacttggtcagtattttcaaaagctgggtcagtgttcagcacgagtttctataaacacagtcaacttgacagttggccctcaggtcatggaagtgattgtctttcgaagacacggccgggcatacattcccatctccaaagtgaaagacgtgtatgtgataacagatcagatccctatattcgtgaccatgtaccagaagaatgaccggaactcgtctgatgaaaccttcctcagagacctccccattttcttcgatgtcctcattcacgatcccagtcatttcctcaactactctgccatttcctacaagtggaactttggggacaacactggcctgtttgtctccaacaatcacactttgaatcacacgtatgtgctcaatggaaccttcaactttaacctcaccgtgcaaactgcagtgccgggaccatgcccctcacccacaccttcgccttcttcttcgacttctccttcgcctgcatcttcgccttcacccacattatcaacacctagtccctctttaatgcctactggctacaaatccatggagctgagtgacatttccaatgaaaactgccgaataaacagatatggttacttcagagccaccatcacaattgtagatggaatcctagaagtcaacatcatccaggtagcagatgtcccaatccccacactgcagcctgacaactcactgatggacttcattgtgacctgcaaaggggccactcccacggaagcctgtacgatcatctctgaccccacctgccagatcgcccagaacagggtgtgcagcccggtggctgtggatgagctgtgcctcctgtccgtgaggagagccttcaatgggtccggcacgtactgtgtgaatttcactctgggagacgatgcaagcctggccctcaccagcgccctgatctctatccctggcaaagacctaggctcccctctgagaacagtgaat

SEQ ID NO: 221 - protein, 516 aa, Artificial Sequence
MECLYYFLGFLLLAARLPLDAAKRFHDVLGNERPSAYMREHNQLNGWSSDENDWNEKLYPVWKRGDMRWKNSWKGGRVQAVLTSDSPALVGSNITFAVNLIFPRCQKEDANGNIVYEKNCRNEAGLSADPYVYNWTAWSEDSDGENGTGQSHHNVFPDGKPFPHHPGWRRWNFIYVFHTLGQYFQKLGRCSVRVSVNTANVTLGPQLMEVTVYRRHGRAYVPIAQVKDVYVVTDQIPVFVTMFQKNDRNSSDETFLKDLPIMFDVLIHDPSHFLNYSTINYKWSFGDNTGLFVSTNHTVNHTYVLNGTFSLNLTVKAAAPGPCPPPPPPPRPSKPTPSLATTLKSYDSNTPGPAGDNPLELSRIPDENCQINRYGHFQATITIVEGILEVNIIQMTDVLMPVPWPESSLIDFVVTCQGSIPTEVCTIISDPTCEITQNTVCSPVDVDEMCLLTVRRTFNGSGTYCVNLTLGDDTSLALTSTLISVPDRDPASPLRMANEFDYKDDDDKLEHHHHHH

SEQ ID NO: 222 - DNA, 1551 bp, Artificial Sequence
  source 1..1551: mol_type = other DNA
atggaatgtctctactatttcctgggatttctgctcctggctgcaagattgccacttgatgccgccaaacgatttcatgatgtgctgggcaatgaaagaccttctgcttacatgagggagcacaatcaattaaatggctggtcttctgatgaaaatgactggaatgaaaaactctacccagtgtggaagcggggagacatgaggtggaaaaactcctggaagggaggccgtgtgcaggcggtcctgaccagtgactcaccagccctcgtgggctcaaatataacatttgcggtgaacctgatattccctagatgccaaaaggaagatgccaatggcaacatagtctatgagaagaactgcagaaatgaggctggtttatctgctgatccgtatgtttacaactggacagcatggtcagaggacagtgacggggaaaatggcaccggccaaagccatcataacgtcttccctgatgggaaaccttttcctcaccaccccggatggagaagatggaatttcatctacgtcttccacacacttggtcagtatttccagaaattgggacgatgttcagtgagagtttctgtgaacacagccaatgtgacacttgggcctcaactcatggaagtgactgtctacagaagacatggacgggcatatgttcccatcgcacaagtgaaagatgtgtacgtggtaacagatcagattcctgtgtttgtgactatgttccagaagaacgatcgaaattcatccgacgaaaccttcctcaaagatctccccattatgtttgatgtcctgattcatgatcctagccacttcctcaattattctaccattaactacaagtggagcttcggggataatactggcctgtttgtttccaccaatcatactgtgaatcacacgtatgtgctcaatggaaccttcagccttaacctcactgtgaaagctgcagcaccaggaccttgtccgccaccgccaccaccacccagaccttcaaaacccaccccttctttagcaactactctaaaatcttatgattcaaacaccccaggacctgctggtgacaaccccctggagctgagtaggattcctgatgaaaactgccagattaacagatatggccactttcaagccaccatcacaattgtagagggaatcttagaggttaacatcatccagatgacagacgtcctgatgccggtgccatggcctgaaagctccctaatagactttgtcgtgacctgccaagggagcattcccacggaggtctgtaccatcatttctgaccccacctgcgagatcacccagaacacagtctgcagccctgtggatgtggatgagatgtgtctgctgactgtgagacgaaccttcaatgggtctgggacgtactgtgtgaacctcaccctgggggatgacacaagcctggctctcacgagcaccctgatttctgttcctgacagagacccagcctcgcctttaaggatggcaaacgaattcgattataaggatgacgatgacaagctcgagcatcaccaccatcaccactaa

SEQ ID NO: 223 - protein, 520 aa, Artificial Sequence
MESLCGVLGFLLLAAGLPLQAAKRFRDVLGHEQYPDHMREHNQLRGWSSDENEWDEHLYPVWRRGDGRWKDSWEGGRVQAVLTSDSPALVGSNITFVVNLVFPRCQKEDANGNIVYEKNCRNDLGLTSDLHVYNWTAGADDGDWEDGTSRSQHLRFPDRRPFPRPHGWKKWSFVYVFHTLGQYFQKLGRCSARVSINTVNLTAGPQVMEVTVFRRYGRAYIPISKVKDVYVITDQIPVFVTMSQKNDRNLSDEIFLRDLPIVFDVLIHDPSHFLNDSAISYKWNFGDNTGLFVSNNHTLNHTYVLNGTFNLNLTVQTAVPGPCPPPSPSTPPPPSTPPSPPPSPLPTLSTPSPSLMPTGYKSMELSDISNENCRINRYGYFRATITIVEGILEVSIMQIADVPMPTPQPANSLMDFTVTCKGATPMEACTIISDPTCQIAQNRVCSPVAVDGLCLLSVRRAFNGSGTYCVNFTLGDDASLALTSTLISIPGKDPDSPLRAVNEFDYKDDDDKLEHHHHHH

SEQ ID NO: 224 - DNA, 1563 bp, Artificial Sequence
  source 1..1563: mol_type = other DNA
atggaaagtctctgcggggtcctgggatttctgctgctggctgcaggactgcctctccaggctgccaagcgatttcgtgatgtgctgggccatgaacagtatcccgatcacatgagagagcacaaccaattacgtggctggtcttcggatgaaaatgaatgggatgaacacctgtatccagtgtggaggaggggagacggcaggtggaaggactcctgggaaggaggccgtgtgcaggcagtcctgaccagtgactcaccggctctggtgggttccaatatcacttttgtggtgaacctggtgttccccagatgccagaaggaagatgctaatggcaatatcgtctatgagaagaactgcaggaatgatttgggactgacatctgacctgcatgtctacaactggactgcaggggcagatgatggtgactgggaagatggcaccagccgaagccagcatctcaggttcccggacaggaggcccttccctcgcccccatggatggaagaaatggagctttgtctacgtctttcacacacttggccagtatttccaaaaactgggtcggtgttcagcacgggtttctataaacacagtcaacttgacagctggccctcaggtcatggaagtgactgtctttcgaagatacggccgggcatacattcccatctcgaaggtgaaagatgtgtatgtgataacagatcagatccctgtattcgtgaccatgtcccagaagaatgacaggaacttgtctgatgagatcttcctcagagacctccccatcgtcttcgatgtcctcattcatgatcccagccacttcctcaacgactctgccatttcctacaagtggaactttggggacaacactggcctgtttgtctccaacaatcacactttgaatcacacttatgtgctcaatggaaccttcaaccttaacctcaccgtgcaaactgcagtgcccgggccatgccctcccccttcgccttcgactccgcctccaccttcaactccgccctcacctccgccctcacctctgcccacattatcaacacctagcccctctttaatgcctactggttacaaatccatggagctgagtgacatttccaatgaaaactgccgaataaacagatatggctacttcagagccaccatcacaattgtagaggggatcctggaagtcagcatcatgcagatagcagatgtccccatgcccacaccgcagcctgccaactccctgatggacttcactgtgacctgcaaaggggccacccccatggaagcctgtacgatcatctccgaccccacctgccagatcgcccagaaccgggtctgcagccctgtggctgtggatgggctgtgcctgctgtctgtgagaagagccttcaatgggtctggcacctactgtgtgaatttcactctgggagatgatgcaagcctggccctcaccagcaccctgatctctatccctggcaaagacccagactcccctctgagagcagtgaatgaattcgattataaggatgacgatgacaagctcgagcatcaccaccatcaccactaa

SEQ ID NO: 225 - protein, 518 aa, Artificial Sequence
MESLCGVLVFLLLAAGLPLQAAKRFRDVLGHEQYPDHMRENNQLRGWSSDENEWDEQLYPVWRRGEGRWKDSWEGGRVQAALTSDSPALVGSNITFVVNLVFPRCQKEDANGNIVYERNCRSDLELASDPYVYNWTTGADDEDWEDNTSQGQHLRFPDGKPFPRPHGRKKWNFVYVFHTLGQYFQKLGQCSARVSINTVNLTVGPQVMEVIVFRRHGRAYIPISKVKDVYVITDQIPIFVTMYQKNDRNSSDETFLRDLPIFFDVLIHDPSHFLNYSAISYKWNFGDNTGLFVSNNHTLNHTYVLNGTFNFNLTVQTAVPGPCPSPTPSPSSSTSPSPASSPSPTLSTPSPSLMPTGYKSMELSDISNENCRINRYGYFRATITIVDGILEVNIIQVADVPIPTLQPDNSLMDFIVTCKGATPTEACTIISDPTCQIAQNRVCSPVAVDELCLLSVRRAFNGSGTYCVNFTLGDDASLALTSALISIPGKDLGSPLRTVNEFDYKDDDDKLEHHHHHH

SEQ ID NO: 226 - DNA, 1557 bp, Artificial Sequence
  source 1..1557: mol_type = other DNA
atggaaagtctctgcggggtcctggtatttctgctgctggctgcaggactgccgctccaggcggccaagcggttccgtgatgtgctgggccatgagcagtatccggatcacatgagggagaacaaccaattacgtggctggtcttcagatgaaaatgaatgggatgaacagctgtatccagtgtggaggaggggagagggcagatggaaggactcctgggaaggaggccgtgtgcaggcagccctaaccagtgattcaccggccttggtgggttccaatatcaccttcgtagtgaacctggtgttccccagatgccagaaggaagatgccaacggcaatatcgtctatgagaggaactgcagaagtgatttggagctggcttctgacccgtatgtctacaactggaccacaggggcagacgatgaggactgggaagacaacaccagccaaggccagcacctcaggttccccgacgggaagcccttccctcgcccccacggacggaagaaatggaacttcgtctacgtcttccacacacttggtcagtattttcaaaagctgggtcagtgttcagcacgagtttctataaacacagtcaacttgacagttggccctcaggtcatggaagtgattgtctttcgaagacacggccgggcatacattcccatctccaaagtgaaagacgtgtatgtgataacagatcagatccctatattcgtgaccatgtaccagaagaatgaccggaactcgtctgatgaaaccttcctcagagacctccccattttcttcgatgtcctcattcacgatcccagtcatttcctcaactactctgccatttcctacaagtggaactttggggacaacactggcctgtttgtctccaacaatcacactttgaatcacacgtatgtgctcaatggaaccttcaactttaacctcaccgtgcaaactgcagtgccgggaccatgcccctcacccacaccttcgccttcttcttcgacttctccttcgcctgcatcttcgccttcacccacattatcaacacctagtccctctttaatgcctactggctacaaatccatggagctgagtgacatttccaatgaaaactgccgaataaacagatatggttacttcagagccaccatcacaattgtagatggaatcctagaagtcaacatcatccaggtagcagatgtcccaatccccacactgcagcctgacaactcactgatggacttcattgtgacctgcaaaggggccactcccacggaagcctgtacgatcatctctgaccccacctgccagatcgcccagaacagggtgtgcagcccggtggctgtggatgagctgtgcctcctgtccgtgaggagagccttcaatgggtccggcacgtactgtgtgaatttcactctgggagacgatgcaagcctggccctcaccagcgccctgatctctatccctggcaaagacctaggctcccctctgagaacagtgaatgaattcgattataaggatgacgatgacaagctcgagcatcaccaccatcaccactaa

SEQ ID NO: 227 - protein, 269 aa, Artificial Sequence
MECLYYFLGFLLLAARLPLDAAKRFHDVLGNERPSAYMREHNQLNGWSSDENDWNEKLYPVWKRGDMRWKNSWKGGRVQAVLTSDSPALVGSNITFAVNLIFPRCQKEDANGNIVYEKNCRNEAGLSADPYVYNWTAWSEDSDGENGTGQSHHNVFPDGKPFPHHPGWRRWNFIYVFHTLGQYFQKLGRCSVRVSVNTANVTLGPQLMEVTVYRRHGRAYVPIAQVKDVYVVTDQIPVFVTMFQKNDRNSSEFDYKDDDDKLEHHHHHH

SEQ ID NO: 228 - DNA, 807 bp, Artificial Sequence
  source 1..807: mol_type = other DNA
atggaatgtctctactatttcctgggatttctgctcctggctgcaagattgccacttgatgccgccaaacgatttcatgatgtgctgggcaatgaaagaccttctgcttacatgagggagcacaatcaattaaatggctggtcttctgatgaaaatgactggaatgaaaaactctacccagtgtggaagcggggagacatgaggtggaaaaactcctggaagggaggccgtgtgcaggcggtcctgaccagtgactcaccagccctcgtgggctcaaatataacatttgcggtgaacctgatattccctagatgccaaaaggaagatgccaatggcaacatagtctatgagaagaactgcagaaatgaggctggtttatctgctgatccgtatgtttacaactggacagcatggtcagaggacagtgacggggaaaatggcaccggccaaagccatcataacgtcttccctgatgggaaaccttttcctcaccaccccggatggagaagatggaatttcatctacgtcttccacacacttggtcagtatttccagaaattgggacgatgttcagtgagagtttctgtgaacacagccaatgtgacacttgggcctcaactcatggaagtgactgtctacagaagacatggacgggcatatgttcccatcgcacaagtgaaagatgtgtacgtggtaacagatcagattcctgtgtttgtgactatgttccagaagaacgatcgaaattcatccgaattcgattataaggatgacgatgacaagctcgagcatcaccaccatcaccac

SEQ ID NO: 229 - protein, 339 aa, Artificial Sequence
MECLYYFLGFLLLAARLPLDAAKRFHDVLGNERPSAYMREHNQLNGWSSDENDWNEKLYPVWKRGDMRWKNSWKGGRVQAVLTSDSPALVGSNITFAVNLIFPRCQKEDANGNIVYEKNCRNEAGLSADPYVYNWTAWSEDSDGENGTGQSHHNVFPDGKPFPHHPGWRRWNFIYVFHTLGQYFQKLGRCSVRVSVNTANVTLGPQLMEVTVYRRHGRAYVPIAQVKDVYVVTDQIPVFVTMFQKNDRNSSDETFLKDLPIMFDVLIHDPSHFLNYSTINYKWSFGDNTGLFVSTNHTVNHTYVLNGTFSLNLTVKAAAPGEFDYKDDDDKLEHHHHHH

SEQ ID NO: 230 - DNA, 1020 bp, Artificial Sequence
  source 1..1020: mol_type = other DNA
atggaatgtctctactatttcctgggatttctgctcctggctgcaagattgccacttgatgccgccaaacgatttcatgatgtgctgggcaatgaaagaccttctgcttacatgagggagcacaatcaattaaatggctggtcttctgatgaaaatgactggaatgaaaaactctacccagtgtggaagcggggagacatgaggtggaaaaactcctggaagggaggccgtgtgcaggcggtcctgaccagtgactcaccagccctcgtgggctcaaatataacatttgcggtgaacctgatattccctagatgccaaaaggaagatgccaatggcaacatagtctatgagaagaactgcagaaatgaggctggtttatctgctgatccgtatgtttacaactggacagcatggtcagaggacagtgacggggaaaatggcaccggccaaagccatcataacgtcttccctgatgggaaaccttttcctcaccaccccggatggagaagatggaatttcatctacgtcttccacacacttggtcagtatttccagaaattgggacgatgttcagtgagagtttctgtgaacacagccaatgtgacacttgggcctcaactcatggaagtgactgtctacagaagacatggacgggcatatgttcccatcgcacaagtgaaagatgtgtacgtggtaacagatcagattcctgtgtttgtgactatgttccagaagaacgatcgaaattcatccgacgaaaccttcctcaaagatctccccattatgtttgatgtcctgattcatgatcctagccacttcctcaattattctaccattaactacaagtggagcttcggggataatactggcctgtttgtttccaccaatcatactgtgaatcacacgtatgtgctcaatggaaccttcagccttaacctcactgtgaaagctgcagcaccaggagaattcgattataaggatgacgatgacaagctcgagcatcaccaccatcaccactaa

SEQ ID NO: 231 - protein, 393 aa, Artificial Sequence
MECLYYFLGFLLLAARLPLDAAKRFHDVLGNERPSAYMREHNQLNGWSSDENDWNEKLYPVWKRGDMRWKNSWKGGRVQAVLTSDSPALVGSNITFAVNLIFPRCQKEDANGNIVYEKNCRNEAGLSADPYVYNWTAWSEDSDGENGTGQSHHNVFPDGKPFPHHPGWRRWNFIYVFHTLGQYFQKLGRCSVRVSVNTANVTLGPQLMEVTVYRRHGRAYVPIAQVKDVYVVTDQIPVFVTMFQKNDRNSSDETFLKDLPIMFDVLIHDPSHFLNYSTINYKWSFGDNTGLFVSTNHTVNHTYVLNGTFSLNLTVKAAAPGPCPPPPPPPRPSKPTPSLATTLKSYDSNTPGPAGDNPLELSRIPDENCQINRYGEFDYKDDDDKLEHHHHHH

SEQ ID NO: 232 - DNA, 1182 bp, Artificial Sequence
  source 1..1182: mol_type = other DNA
atggaatgtctctactatttcctgggatttctgctcctggctgcaagattgccacttgatgccgccaaacgatttcatgatgtgctgggcaatgaaagaccttctgcttacatgagggagcacaatcaattaaatggctggtcttctgatgaaaatgactggaatgaaaaactctacccagtgtggaagcggggagacatgaggtggaaaaactcctggaagggaggccgtgtgcaggcggtcctgaccagtgactcaccagccctcgtgggctcaaatataacatttgcggtgaacctgatattccctagatgccaaaaggaagatgccaatggcaacatagtctatgagaagaactgcagaaatgaggctggtttatctgctgatccgtatgtttacaactggacagcatggtcagaggacagtgacggggaaaatggcaccggccaaagccatcataacgtcttccctgatgggaaaccttttcctcaccaccccggatggagaagatggaatttcatctacgtcttccacacacttggtcagtatttccagaaattgggacgatgttcagtgagagtttctgtgaacacagccaatgtgacacttgggcctcaactcatggaagtgactgtctacagaagacatggacgggcatatgttcccatcgcacaagtgaaagatgtgtacgtggtaacagatcagattcctgtgtttgtgactatgttccagaagaacgatcgaaattcatccgacgaaaccttcctcaaagatctccccattatgtttgatgtcctgattcatgatcctagccacttcctcaattattctaccattaactacaagtggagcttcggggataatactggcctgtttgtttccaccaatcatactgtgaatcacacgtatgtgctcaatggaaccttcagccttaacctcactgtgaaagctgcagcaccaggaccttgtccgccaccgccaccaccacccagaccttcaaaacccaccccttctttagcaactactctaaaatcttatgattcaaacaccccaggacctgctggtgacaaccccctggagctgagtaggattcctgatgaaaactgccagattaacagatatggcgaattcgattataaggatgacgatgacaagctcgagcatcaccaccatcaccactaa

SEQ ID NO: 233 - protein, 436 aa, Artificial Sequence
MECLYYFLGFLLLAARLPLDAAKRFHDVLGNERPSAYMREHNQLNGWSSDENDWNEKLYPVWKRGDMRWKNSWKGGRVQAVLTSDSPALVGSNITFAVNLIFPRCQKEDANGNIVYEKNCRNEAGLSADPYVYNWTAWSEDSDGENGTGQSHHNVFPDGKPFPHHPGWRRWNFIYVFHTLGQYFQKLGRCSVRVSVNTANVTLGPQLMEVTVYRRHGRAYVPIAQVKDVYVVTDQIPVFVTMFQKNDRNSSDETFLKDLPIMFDVLIHDPSHFLNYSTINYKWSFGDNTGLFVSTNHTVNHTYVLNGTFSLNLTVKAAAPGPCPPPPPPPRPSKPTPSLATTLKSYDSNTPGPAGDNPLELSRIPDENCQINRYGHFQATITIVEGILEVNIIQMTDVLMPVPWPESSLIDFVVTCQGEFDYKDDDDKLEHHHHHH

SEQ ID NO: 234 - DNA, 1311 bp, Artificial Sequence
  source 1..1311: mol_type = other DNA
atggaatgtctctactatttcctgggatttctgctcctggctgcaagattgccacttgatgccgccaaacgatttcatgatgtgctgggcaatgaaagaccttctgcttacatgagggagcacaatcaattaaatggctggtcttctgatgaaaatgactggaatgaaaaactctacccagtgtggaagcggggagacatgaggtggaaaaactcctggaagggaggccgtgtgcaggcggtcctgaccagtgactcaccagccctcgtgggctcaaatataacatttgcggtgaacctgatattccctagatgccaaaaggaagatgccaatggcaacatagtctatgagaagaactgcagaaatgaggctggtttatctgctgatccgtatgtttacaactggacagcatggtcagaggacagtgacggggaaaatggcaccggccaaagccatcataacgtcttccctgatgggaaaccttttcctcaccaccccggatggagaagatggaatttcatctacgtcttccacacacttggtcagtatttccagaaattgggacgatgttcagtgagagtttctgtgaacacagccaatgtgacacttgggcctcaactcatggaagtgactgtctacagaagacatggacgggcatatgttcccatcgcacaagtgaaagatgtgtacgtggtaacagatcagattcctgtgtttgtgactatgttccagaagaacgatcgaaattcatccgacgaaaccttcctcaaagatctccccattatgtttgatgtcctgattcatgatcctagccacttcctcaattattctaccattaactacaagtggagcttcggggataatactggcctgtttgtttccaccaatcatactgtgaatcacacgtatgtgctcaatggaaccttcagccttaacctcactgtgaaagctgcagcaccaggaccttgtccgccaccgccaccaccacccagaccttcaaaacccaccccttctttagcaactactctaaaatcttatgattcaaacaccccaggacctgctggtgacaaccccctggagctgagtaggattcctgatgaaaactgccagattaacagatatggccactttcaagccaccatcacaattgtagagggaatcttagaggttaacatcatccagatgacagacgtcctgatgccggtgccatggcctgaaagctccctaatagactttgtcgtgacctgccaaggggaattcgattataaggatgacgatgacaagctcgagcatcaccaccatcaccactaa

SEQ ID NO: 235 - protein, 465 aa, Artificial Sequence
MECLYYFLGFLLLAARLPLDAAGSGRVQAVLTSDSPALVGSNITFAVNLIFPRCQKEDANGNIVYEKNCRNEAGLSADPYVYNWTAWSEDSDGENGTGQSHHNVFPDGKPFPHHPGWRRWNFIYVFHTLGQYFQKLGRCSVRVSVNTANVTLGPQLMEVTVYRRHGRAYVPIAQVKDVYVVTDQIPVFVTMFQKNDRNSSDETFLKDLPIMFDVLIHDPSHFLNYSTINYKWSFGDNTGLFVSTNHTVNHTYVLNGTFSLNLTVKAAAPGPCPPPPPPPRPSKPTPSLATTLKSYDSNTPGPAGDNPLELSRIPDENCQINRYGHFQATITIVEGILEVNIIQMTDVLMPVPWPESSLIDFVVTCQGSIPTEVCTIISDPTCEITQNTVCSPVDVDEMCLLTVRRTFNGSGTYCVNLTLGDDTSLALTSTLISVPDRDPASPLRMANEFDYKDDDDKLEHHHHHH

SEQ ID NO: 236 - DNA, 1398 bp, Artificial Sequence
  source 1..1398: mol_type = other DNA
atggaatgtctctactatttcctgggatttctgctcctggctgcaagattgccacttgatgccgccggatccggccgtgtgcaggcggtcctgaccagtgactcaccagccctcgtgggctcaaatataacatttgcggtgaacctgatattccctagatgccaaaaggaagatgccaatggcaacatagtctatgagaagaactgcagaaatgaggctggtttatctgctgatccgtatgtttacaactggacagcatggtcagaggacagtgacggggaaaatggcaccggccaaagccatcataacgtcttccctgatgggaaaccttttcctcaccaccccggatggagaagatggaatttcatctacgtcttccacacacttggtcagtatttccagaaattgggacgatgttcagtgagagtttctgtgaacacagccaatgtgacacttgggcctcaactcatggaagtgactgtctacagaagacatggacgggcatatgttcccatcgcacaagtgaaagatgtgtacgtggtaacagatcagattcctgtgtttgtgactatgttccagaagaacgatcgaaattcatccgacgaaaccttcctcaaagatctccccattatgtttgatgtcctgattcatgatcctagccacttcctcaattattctaccattaactacaagtggagcttcggggataatactggcctgtttgtttccaccaatcatactgtgaatcacacgtatgtgctcaatggaaccttcagccttaacctcactgtgaaagctgcagcaccaggaccttgtccgccaccgccaccaccacccagaccttcaaaacccaccccttctttagcaactactctaaaatcttatgattcaaacaccccaggacctgctggtgacaaccccctggagctgagtaggattcctgatgaaaactgccagattaacagatatggccactttcaagccaccatcacaattgtagagggaatcttagaggttaacatcatccagatgacagacgtcctgatgccggtgccatggcctgaaagctccctaatagactttgtcgtgacctgccaagggagcattcccacggaggtctgtaccatcatttctgaccccacctgcgagatcacccagaacacagtctgcagccctgtggatgtggatgagatgtgtctgctgactgtgagacgaaccttcaatgggtctgggacatactgtgtgaacctcaccctgggggatgacacaagcctggctctcacgagcaccctgatttctgttcctgacagagacccagcctcgcctttaaggatggcaaacgaattcgattataaggatgacgatgacaagctcgagcatcaccaccatcaccactaa

SEQ ID NO: 237 - protein, 430 aa, Artificial Sequence
MECLYYFLGFLLLAARLPLDAAKRFHDVLGNERPSAYMREHNQLNGWSSDENDWNEKLYPVWKRGDMRWKNSWKGGRVQAVLTSDSPALVGSNITFAVNLIFPRCQKEDANGNIVYEKNCRNEAGLSADPYVYNWTAWSEDSDGENGTGQSHHNVFPDGKPFPHHPGWRRWNFIYVFHTLGQYFQKLGRCSVRVSVNTANVTLGPQLMEVTVYRRHGRAYVPIAQVKDVYVVTDQIPVFVTMFQKNDRNSSDETFLKDLPIMFDVLIHDPSHFLNYSTINYKWSFGDNTGLFVSTNHTVNHTYVLNGTFSLNLTVKAAAPGPCPPPPPPPRPSKPTPSLATTLKSYDSNTPGPAGDNPLELSRIPDENCQINRYGHFQATITIVEGILEVNIIQMTDVLMPVPWPESSLIDFEFDYKDDDDKLEHHHHHH

SEQ ID NO: 238 - DNA, 1293 bp, Artificial Sequence
  source 1..1293: mol_type = other DNA
atggaatgtctctactatttcctgggatttctgctcctggctgcaagattgccacttgatgccgccaaacgatttcatgatgtgctgggcaatgaaagaccttctgcttacatgagggagcacaatcaattaaatggctggtcttctgatgaaaatgactggaatgaaaaactctacccagtgtggaagcggggagacatgaggtggaaaaactcctggaagggaggccgtgtgcaggcggtcctgaccagtgactcaccagccctcgtgggctcaaatataacatttgcggtgaacctgatattccctagatgccaaaaggaagatgccaatggcaacatagtctatgagaagaactgcagaaatgaggctggtttatctgctgatccgtatgtttacaactggacagcatggtcagaggacagtgacggggaaaatggcaccggccaaagccatcataacgtcttccctgatgggaaaccttttcctcaccaccccggatggagaagatggaatttcatctacgtcttccacacacttggtcagtatttccagaaattgggacgatgttcagtgagagtttctgtgaacacagccaatgtgacacttgggcctcaactcatggaagtgactgtctacagaagacatggacgggcatatgttcccatcgcacaagtgaaagatgtgtacgtggtaacagatcagattcctgtgtttgtgactatgttccagaagaacgatcgaaattcatccgacgaaaccttcctcaaagatctccccattatgtttgatgtcctgattcatgatcctagccacttcctcaattattctaccattaactacaagtggagcttcggggataatactggcctgtttgtttccaccaatcatactgtgaatcacacgtatgtgctcaatggaaccttcagccttaacctcactgtgaaagctgcagcaccaggaccttgtccgccaccgccaccaccacccagaccttcaaaacccaccccttctttagcaactactctaaaatcttatgattcaaacaccccaggacctgctggtgacaaccccctggagctgagtaggattcctgatgaaaactgccagattaacagatatggccactttcaagccaccatcacaattgtagagggaatcttagaggttaacatcatccagatgacagacgtcctgatgccggtgccatggcctgaaagctccctaatagactttgaattcgattataaggatgacgatgacaagctcgagcatcaccaccatcaccactaa

SEQ ID NO: 239 - protein, 424 aa, Artificial Sequence
MECLYYFLGFLLLAARLPLDAAKRFHDVLGNERPSAYMREHNQLNGWSSDENDWNEKLYPVWKRGDMRWKNSWKGGRVQAVLTSDSPALVGSNITFAVNLIFPRCQKEDANGNIVYEKNCRNEAGLSADPYVYNWTAWSEDSDGENGTGQSHHNVFPDGKPFPHHPGWRRWNFIYVFHTLGQYFQKLGRCSVRVSVNTANVTLGPQLMEVTVYRRHGRAYVPIAQVKDVYVVTDQIPVFVTMFQKNDRNSSDETFLKDLPIMFDVLIHDPSHFLNYSTINYKWSFGDNTGLFVSTNHTVNHTYVLNGTFSLNLTVKAAAPGPCPPPPPPPRPSKPTPSLATTLKSYDSNTPGPAGDNPLELSRIPDENCQINRYGHFQATITIVEGILEVNIIQMTDVLMPVPWPEEFDYKDDDDKLEHHHHHH

SEQ ID NO: 240 - DNA, 1275 bp, Artificial Sequence
  source 1..1275: mol_type = other DNA
atggaatgtctctactatttcctgggatttctgctcctggctgcaagattgccacttgatgccgccaaacgatttcatgatgtgctgggcaatgaaagaccttctgcttacatgagggagcacaatcaattaaatggctggtcttctgatgaaaatgactggaatgaaaaactctacccagtgtggaagcggggagacatgaggtggaaaaactcctggaagggaggccgtgtgcaggcggtcctgaccagtgactcaccagccctcgtgggctcaaatataacatttgcggtgaacctgatattccctagatgccaaaaggaagatgccaatggcaacatagtctatgagaagaactgcagaaatgaggctggtttatctgctgatccgtatgtttacaactggacagcatggtcagaggacagtgacggggaaaatggcaccggccaaagccatcataacgtcttccctgatgggaaaccttttcctcaccaccccggatggagaagatggaatttcatctacgtcttccacacacttggtcagtatttccagaaattgggacgatgttcagtgagagtttctgtgaacacagccaatgtgacacttgggcctcaactcatggaagtgactgtctacagaagacatggacgggcatatgttcccatcgcacaagtgaaagatgtgtacgtggtaacagatcagattcctgtgtttgtgactatgttccagaagaacgatcgaaattcatccgacgaaaccttcctcaaagatctccccattatgtttgatgtcctgattcatgatcctagccacttcctcaattattctaccattaactacaagtggagcttcggggataatactggcctgtttgtttccaccaatcatactgtgaatcacacgtatgtgctcaatggaaccttcagccttaacctcactgtgaaagctgcagcaccaggaccttgtccgccaccgccaccaccacccagaccttcaaaacccaccccttctttagcaactactctaaaatcttatgattcaaacaccccaggacctgctggtgacaaccccctggagctgagtaggattcctgatgaaaactgccagattaacagatatggccactttcaagccaccatcacaattgtagagggaatcttagaggttaacatcatccagatgacagacgtcctgatgccggtgccatggcctgaagaattcgattataaggatgacgatgacaagctcgagcatcaccaccatcaccactaa

SEQ ID NO: 241 - protein, 418 aa, Artificial Sequence
MECLYYFLGFLLLAARLPLDAAKRFHDVLGNERPSAYMREHNQLNGWSSDENDWNEKLYPVWKRGDMRWKNSWKGGRVQAVLTSDSPALVGSNITFAVNLIFPRCQKEDANGNIVYEKNCRNEAGLSADPYVYNWTAWSEDSDGENGTGQSHHNVFPDGKPFPHHPGWRRWNFIYVFHTLGQYFQKLGRCSVRVSVNTANVTLGPQLMEVTVYRRHGRAYVPIAQVKDVYVVTDQIPVFVTMFQKNDRNSSDETFLKDLPIMFDVLIHDPSHFLNYSTINYKWSFGDNTGLFVSTNHTVNHTYVLNGTFSLNLTVKAAAPGPCPPPPPPPRPSKPTPSLATTLKSYDSNTPGPAGDNPLELSRIPDENCQINRYGHFQATITIVEGILEVNIIQMTDVLMEFDYKDDDDKLEHHHHHH

SEQ ID NO: 242 - DNA, 1257 bp, Artificial Sequence
  source 1..1257: mol_type = other DNA
atggaatgtctctactatttcctgggatttctgctcctggctgcaagattgccacttgatgccgccaaacgatttcatgatgtgctgggcaatgaaagaccttctgcttacatgagggagcacaatcaattaaatggctggtcttctgatgaaaatgactggaatgaaaaactctacccagtgtggaagcggggagacatgaggtggaaaaactcctggaagggaggccgtgtgcaggcggtcctgaccagtgactcaccagccctcgtgggctcaaatataacatttgcggtgaacctgatattccctagatgccaaaaggaagatgccaatggcaacatagtctatgagaagaactgcagaaatgaggctggtttatctgctgatccgtatgtttacaactggacagcatggtcagaggacagtgacggggaaaatggcaccggccaaagccatcataacgtcttccctgatgggaaaccttttcctcaccaccccggatggagaagatggaatttcatctacgtcttccacacacttggtcagtatttccagaaattgggacgatgttcagtgagagtttctgtgaacacagccaatgtgacacttgggcctcaactcatggaagtgactgtctacagaagacatggacgggcatatgttcccatcgcacaagtgaaagatgtgtacgtggtaacagatcagattcctgtgtttgtgactatgttccagaagaacgatcgaaattcatccgacgaaaccttcctcaaagatctccccattatgtttgatgtcctgattcatgatcctagccacttcctcaattattctaccattaactacaagtggagcttcggggataatactggcctgtttgtttccaccaatcatactgtgaatcacacgtatgtgctcaatggaaccttcagccttaacctcactgtgaaagctgcagcaccaggaccttgtccgccaccgccaccaccacccagaccttcaaaacccaccccttctttagcaactactctaaaatcttatgattcaaacaccccaggacctgctggtgacaaccccctggagctgagtaggattcctgatgaaaactgccagattaacagatatggccactttcaagccaccatcacaattgtagagggaatcttagaggttaacatcatccagatgacagacgtcctgatggaattcgattataaggatgacgatgacaagctcgagcatcaccaccatcaccactaa

SEQ ID NO: 243 - protein, 412 aa, Artificial Sequence
MECLYYFLGFLLLAARLPLDAAKRFHDVLGNERPSAYMREHNQLNGWSSDENDWNEKLYPVWKRGDMRWKNSWKGGRVQAVLTSDSPALVGSNITFAVNLIFPRCQKEDANGNIVYEKNCRNEAGLSADPYVYNWTAWSEDSDGENGTGQSHHNVFPDGKPFPHHPGWRRWNFIYVFHTLGQYFQKLGRCSVRVSVNTANVTLGPQLMEVTVYRRHGRAYVPIAQVKDVYVVTDQIPVFVTMFQKNDRNSSDETFLKDLPIMFDVLIHDPSHFLNYSTINYKWSFGDNTGLFVSTNHTVNHTYVLNGTFSLNLTVKAAAPGPCPPPPPPPRPSKPTPSLATTLKSYDSNTPGPAGDNPLELSRIPDENCQINRYGHFQATITIVEGILEVNIIQEFDYKDDDDKLEHHHHHH

SEQ ID NO: 244 - DNA, 1239 bp, Artificial Sequence
  source 1..1239: mol_type = other DNA
atggaatgtctctactatttcctgggatttctgctcctggctgcaagattgccacttgatgccgccaaacgatttcatgatgtgctgggcaatgaaagaccttctgcttacatgagggagcacaatcaattaaatggctggtcttctgatgaaaatgactggaatgaaaaactctacccagtgtggaagcggggagacatgaggtggaaaaactcctggaagggaggccgtgtgcaggcggtcctgaccagtgactcaccagccctcgtgggctcaaatataacatttgcggtgaacctgatattccctagatgccaaaaggaagatgccaatggcaacatagtctatgagaagaactgcagaaatgaggctggtttatctgctgatccgtatgtttacaactggacagcatggtcagaggacagtgacggggaaaatggcaccggccaaagccatcataacgtcttccctgatgggaaaccttttcctcaccaccccggatggagaagatggaatttcatctacgtcttccacacacttggtcagtatttccagaaattgggacgatgttcagtgagagtttctgtgaacacagccaatgtgacacttgggcctcaactcatggaagtgactgtctacagaagacatggacgggcatatgttcccatcgcacaagtgaaagatgtgtacgtggtaacagatcagattcctgtgtttgtgactatgttccagaagaacgatcgaaattcatccgacgaaaccttcctcaaagatctccccattatgtttgatgtcctgattcatgatcctagccacttcctcaattattctaccattaactacaagtggagcttcggggataatactggcctgtttgtttccaccaatcatactgtgaatcacacgtatgtgctcaatggaaccttcagccttaacctcactgtgaaagctgcagcaccaggaccttgtccgccaccgccaccaccacccagaccttcaaaacccaccccttctttagcaactactctaaaatcttatgattcaaacaccccaggacctgctggtgacaaccccctggagctgagtaggattcctgatgaaaactgccagattaacagatatggccactttcaagccaccatcacaattgtagagggaatcttagaggttaacatcatccaggaattcgattataaggatgacgatgacaagctcgagcatcaccaccatcaccactaa

SEQ ID NO: 245 - protein, 406 aa, Artificial Sequence
MECLYYFLGFLLLAARLPLDAAKRFHDVLGNERPSAYMREHNQLNGWSSDENDWNEKLYPVWKRGDMRWKNSWKGGRVQAVLTSDSPALVGSNITFAVNLIFPRCQKEDANGNIVYEKNCRNEAGLSADPYVYNWTAWSEDSDGENGTGQSHHNVFPDGKPFPHHPGWRRWNFIYVFHTLGQYFQKLGRCSVRVSVNTANVTLGPQLMEVTVYRRHGRAYVPIAQVKDVYVVTDQIPVFVTMFQKNDRNSSDETFLKDLPIMFDVLIHDPSHFLNYSTINYKWSFGDNTGLFVSTNHTVNHTYVLNGTFSLNLTVKAAAPGPCPPPPPPPRPSKPTPSLATTLKSYDSNTPGPAGDNPLELSRIPDENCQINRYGHFQATITIVEGILEFDYKDDDDKLEHHHHHH

SEQ ID NO: 246 - DNA, 1221 bp, Artificial Sequence
  source 1..1221: mol_type = other DNA
atggaatgtctctactatttcctgggatttctgctcctggctgcaagattgccacttgatgccgccaaacgatttcatgatgtgctgggcaatgaaagaccttctgcttacatgagggagcacaatcaattaaatggctggtcttctgatgaaaatgactggaatgaaaaactctacccagtgtggaagcggggagacatgaggtggaaaaactcctggaagggaggccgtgtgcaggcggtcctgaccagtgactcaccagccctcgtgggctcaaatataacatttgcggtgaacctgatattccctagatgccaaaaggaagatgccaatggcaacatagtctatgagaagaactgcagaaatgaggctggtttatctgctgatccgtatgtttacaactggacagcatggtcagaggacagtgacggggaaaatggcaccggccaaagccatcataacgtcttccctgatgggaaaccttttcctcaccaccccggatggagaagatggaatttcatctacgtcttccacacacttggtcagtatttccagaaattgggacgatgttcagtgagagtttctgtgaacacagccaatgtgacacttgggcctcaactcatggaagtgactgtctacagaagacatggacgggcatatgttcccatcgcacaagtgaaagatgtgtacgtggtaacagatcagattcctgtgtttgtgactatgttccagaagaacgatcgaaattcatccgacgaaaccttcctcaaagatctccccattatgtttgatgtcctgattcatgatcctagccacttcctcaattattctaccattaactacaagtggagcttcggggataatactggcctgtttgtttccaccaatcatactgtgaatcacacgtatgtgctcaatggaaccttcagccttaacctcactgtgaaagctgcagcaccaggaccttgtccgccaccgccaccaccacccagaccttcaaaacccaccccttctttagcaactactctaaaatcttatgattcaaacaccccaggacctgctggtgacaaccccctggagctgagtaggattcctgatgaaaactgccagattaacagatatggccactttcaagccaccatcacaattgtagagggaatcttagaattcgattataaggatgacgatgacaagctcgagcatcaccaccatcaccactaa

SEQ ID NO: 247 - protein, 400 aa, Artificial Sequence
MECLYYFLGFLLLAARLPLDAAKRFHDVLGNERPSAYMREHNQLNGWSSDENDWNEKLYPVWKRGDMRWKNSWKGGRVQAVLTSDSPALVGSNITFAVNLIFPRCQKEDANGNIVYEKNCRNEAGLSADPYVYNWTAWSEDSDGENGTGQSHHNVFPDGKPFPHHPGWRRWNFIYVFHTLGQYFQKLGRCSVRVSVNTANVTLGPQLMEVTVYRRHGRAYVPIAQVKDVYVVTDQIPVFVTMFQKNDRNSSDETFLKDLPIMFDVLIHDPSHFLNYSTINYKWSFGDNTGLFVSTNHTVNHTYVLNGTFSLNLTVKAAAPGPCPPPPPPPRPSKPTPSLATTLKSYDSNTPGPAGDNPLELSRIPDENCQINRYGHFQATITEFDYKDDDDKLEHHHHHH

SEQ ID NO: 248 - DNA, 1203 bp, Artificial Sequence
  source 1..1203: mol_type = other DNA
atggaatgtctctactatttcctgggatttctgctcctggctgcaagattgccacttgatgccgccaaacgatttcatgatgtgctgggcaatgaaagaccttctgcttacatgagggagcacaatcaattaaatggctggtcttctgatgaaaatgactggaatgaaaaactctacccagtgtggaagcggggagacatgaggtggaaaaactcctggaagggaggccgtgtgcaggcggtcctgaccagtgactcaccagccctcgtgggctcaaatataacatttgcggtgaacctgatattccctagatgccaaaaggaagatgccaatggcaacatagtctatgagaagaactgcagaaatgaggctggtttatctgctgatccgtatgtttacaactggacagcatggtcagaggacagtgacggggaaaatggcaccggccaaagccatcataacgtcttccctgatgggaaaccttttcctcaccaccccggatggagaagatggaatttcatctacgtcttccacacacttggtcagtatttccagaaattgggacgatgttcagtgagagtttctgtgaacacagccaatgtgacacttgggcctcaactcatggaagtgactgtctacagaagacatggacgggcatatgttcccatcgcacaagtgaaagatgtgtacgtggtaacagatcagattcctgtgtttgtgactatgttccagaagaacgatcgaaattcatccgacgaaaccttcctcaaagatctccccattatgtttgatgtcctgattcatgatcctagccacttcctcaattattctaccattaactacaagtggagcttcggggataatactggcctgtttgtttccaccaatcatactgtgaatcacacgtatgtgctcaatggaaccttcagccttaacctcactgtgaaagctgcagcaccaggaccttgtccgccaccgccaccaccacccagaccttcaaaacccaccccttctttagcaactactctaaaatcttatgattcaaacaccccaggacctgctggtgacaaccccctggagctgagtaggattcctgatgaaaactgccagattaacagatatggccactttcaagccaccatcacagaattcgattataaggatgacgatgacaagctcgagcatcaccaccatcaccactaa

SEQ ID NO: 249 - protein, 252 aa, Artificial Sequence
MECLYYFLGFLLLAARLPLDAAKRFHDVLGNERPSAYMREHNQLNGWSSDENDWNEKLYPVWKRGDMRWKNSWKGGRVQAVLTSDSPALVGSNITFAVNLIFPRCQKEDANGNIVYEKNCRNEAGLSADPYVYNWTAWSEDSDGENGTGQSHHNVFPDGKPFPHHPGWRRWNFIYVFHTLGQYFQKLGRCSVRVSVNTANVTLGPQLMEVTVYRRHGRAYVPIAQVKDVYVVTDEFDYKDDDDKLEHHHHHH

SEQ ID NO: 250 - DNA, 759 bp, Artificial Sequence
  source 1..759: mol_type = other DNA
atggaatgtctctactatttcctgggatttctgctcctggctgcaagattgccacttgatgccgccaaacgatttcatgatgtgctgggcaatgaaagaccttctgcttacatgagggagcacaatcaattaaatggctggtcttctgatgaaaatgactggaatgaaaaactctacccagtgtggaagcggggagacatgaggtggaaaaactcctggaagggaggccgtgtgcaggcggtcctgaccagtgactcaccagccctcgtgggctcaaatataacatttgcggtgaacctgatattccctagatgccaaaaggaagatgccaatggcaacatagtctatgagaagaactgcagaaatgaggctggtttatctgctgatccgtatgtttacaactggacagcatggtcagaggacagtgacggggaaaatggcaccggccaaagccatcataacgtcttccctgatgggaaaccttttcctcaccaccccggatggagaagatggaatttcatctacgtcttccacacacttggtcagtatttccagaaattgggacgatgttcagtgagagtttctgtgaacacagccaatgtgacacttgggcctcaactcatggaagtgactgtctacagaagacatggacgggcatatgttcccatcgcacaagtgaaagatgtgtacgtggtaacagatgaattcgattataaggatgacgatgacaagctcgagcatcaccaccatcaccactaa

SEQ ID NO: 251 - protein, 516 aa, Artificial Sequence
MECLYYFLGFLLLAARLPLDAAKRFHDVLGNERPSAYMREHNQLNGWSSDENDWNEKLYPVWKRGDMRWKNSWKGGRVQAVLTSDSPALVGSNITFAVNLIFPRCQKEDANGNIVYEKNCRNEAGLSADPYVYNWTAWSEDSDGENGTGQSHHNVFPDGKPFPHHPGWRRWNFIYVFHTLGQYFQKLGRCSVRVSVNTANVTLGPQLMEVTVYRRHGRAYVPIAQVKDVYVVTDQIPVFVTMFQANDRNSSDETFLKDLPIMFDVLIHDPSHFLNYSTINYKWSFGDNTGLFVSTNHTVNHTYVLNGTFSLNLTVKAAAPGPCPPPPPPPRPSKPTPSLATTLKSYDSNTPGPAGDNPLELSRIPDENCQINRYGHFQATITIVEGILEVNIIQMTDVLMPVPWPESSLIDFVVTCQGSIPTEVCTIISDPTCEITQNTVCSPVDVDEMCLLTVRRTFNGSGTYCVNLTLGDDTSLALTSTLISVPDRDPASPLRMANEFDYKDDDDKLEHHHHHH

SEQ ID NO: 252 - DNA, 1551 bp, Artificial Sequence
  source 1..1551: mol_type = other DNA
atggaatgtctctactatttcctgggatttctgctcctggctgcaagattgccacttgatgccgccaaacgatttcatgatgtgctgggcaatgaaagaccttctgcttacatgagggagcacaatcaattaaatggctggtcttctgatgaaaatgactggaatgaaaaactctacccagtgtggaagcggggagacatgaggtggaaaaactcctggaagggaggccgtgtgcaggcggtcctgaccagtgactcaccagccctcgtgggctcaaatataacatttgcggtgaacctgatattccctagatgccaaaaggaagatgccaatggcaacatagtctatgagaagaactgcagaaatgaggctggtttatctgctgatccgtatgtttacaactggacagcatggtcagaggacagtgacggggaaaatggcaccggccaaagccatcataacgtcttccctgatgggaaaccttttcctcaccaccccggatggagaagatggaatttcatctacgtcttccacacacttggtcagtatttccagaaattgggacgatgttcagtgagagtttctgtgaacacagccaatgtgacacttgggcctcaactcatggaagtgactgtctacagaagacatggacgggcatatgttcccatcgcacaagtgaaagatgtgtacgtggtaacagatcagattcctgtgtttgtgactatgttccaggcgaacgatcgaaattcatccgacgaaaccttcctcaaagatctccccattatgtttgatgtcctgattcatgatcctagccacttcctcaattattctaccattaactacaagtggagcttcggggataatactggcctgtttgtttccaccaatcatactgtgaatcacacgtatgtgctcaatggaaccttcagccttaacctcactgtgaaagctgcagcaccaggaccttgtccgccaccgccaccaccacccagaccttcaaaacccaccccttctttagcaactactctaaaatcttatgattcaaacaccccaggacctgctggtgacaaccccctggagctgagtaggattcctgatgaaaactgccagattaacagatatggccactttcaagccaccatcacaattgtagagggaatcttagaggttaacatcatccagatgacagacgtcctgatgccggtgccatggcctgaaagctccctaatagactttgtcgtgacctgccaagggagcattcccacggaggtctgtaccatcatttctgaccccacctgcgagatcacccagaacacagtctgcagccctgtggatgtggatgagatgtgtctgctgactgtgagacgaaccttcaatgggtctgggacgtactgtgtgaacctcaccctgggggatgacacaagcctggctctcacgagcaccctgatttctgttcctgacagagacccagcctcgcctttaaggatggcaaacgaattcgattataaggatgacgatgacaagctcgagcatcaccaccatcaccactaa

SEQ ID NO: 253 - protein, 516 aa, Artificial Sequence
MECLYYFLGFLLLAARLPLDAAKRFHDVLGNERPSAYMREHNQLNGWSSDENDWNEKLYPVWKRGDMRWKNSWKGGRVQAVLTSDSPALVGSNITFAVNLIFPRCQKEDANGNIVYEKNCRNEAGLSADPYVYNWTAWSEDSDGENGTGQSHHNVFPDGKPFPHHPGWRRWNFIYVFHTLGQYFQKLGRCSVRVSVNTANVTLGPQLMEVTVYRRHGRAYVPIAQVKDVYVVTDQIPVFVTMFQKNDRNSSAETFLKDLPIMFDVLIHDPSHFLNYSTINYKWSFGDNTGLFVSTNHTVNHTYVLNGTFSLNLTVKAAAPGPCPPPPPPPRPSKPTPSLATTLKSYDSNTPGPAGDNPLELSRIPDENCQINRYGHFQATITIVEGILEVNIIQMTDVLMPVPWPESSLIDFVVTCQGSIPTEVCTIISDPTCEITQNTVCSPVDVDEMCLLTVRRTFNGSGTYCVNLTLGDDTSLALTSTLISVPDRDPASPLRMANEFDYKDDDDKLEHHHHHH

SEQ ID NO: 254 - DNA, 1551 bp, Artificial Sequence
  source 1..1551: mol_type = other DNA
atggaatgtctctactatttcctgggatttctgctcctggctgcaagattgccacttgatgccgccaaacgatttcatgatgtgctgggcaatgaaagaccttctgcttacatgagggagcacaatcaattaaatggctggtcttctgatgaaaatgactggaatgaaaaactctacccagtgtggaagcggggagacatgaggtggaaaaactcctggaagggaggccgtgtgcaggcggtcctgaccagtgactcaccagccctcgtgggctcaaatataacatttgcggtgaacctgatattccctagatgccaaaaggaagatgccaatggcaacatagtctatgagaagaactgcagaaatgaggctggtttatctgctgatccgtatgtttacaactggacagcatggtcagaggacagtgacggggaaaatggcaccggccaaagccatcataacgtcttccctgatgggaaaccttttcctcaccaccccggatggagaagatggaatttcatctacgtcttccacacacttggtcagtatttccagaaattgggacgatgttcagtgagagtttctgtgaacacagccaatgtgacacttgggcctcaactcatggaagtgactgtctacagaagacatggacgggcatatgttcccatcgcacaagtgaaagatgtgtacgtggtaacagatcagattcctgtgtttgtgactatgttccagaagaacgatcgaaattcatccgccgaaaccttcctcaaagatctccccattatgtttgatgtcctgattcatgatcctagccacttcctcaattattctaccattaactacaagtggagcttcggggataatactggcctgtttgtttccaccaatcatactgtgaatcacacgtatgtgctcaatggaaccttcagccttaacctcactgtgaaagctgcagcaccaggaccttgtccgccaccgccaccaccacccagaccttcaaaacccaccccttctttagcaactactctaaaatcttatgattcaaacaccccaggacctgctggtgacaaccccctggagctgagtaggattcctgatgaaaactgccagattaacagatatggccactttcaagccaccatcacaattgtagagggaatcttagaggttaacatcatccagatgacagacgtcctgatgccggtgccatggcctgaaagctccctaatagactttgtcgtgacctgccaagggagcattcccacggaggtctgtaccatcatttctgaccccacctgcgagatcacccagaacacagtctgcagccctgtggatgtggatgagatgtgtctgctgactgtgagacgaaccttcaatgggtctgggacgtactgtgtgaacctcaccctgggggatgacacaagcctggctctcacgagcaccctgatttctgttcctgacagagacccagcctcgcctttaaggatggcaaacgaattcgattataaggatgacgatgacaagctcgagcatcaccaccatcaccactaa

SEQ ID NO: 255 - protein, 516 aa, Artificial Sequence
MECLYYFLGFLLLAARLPLDAAKRFHDVLGNERPSAYMREHNQLNGWSSDENDWNEKLYPVWKRGDMRWKNSWKGGRVQAVLTSDSPALVGSNITFAVNLIFPRCQKEDANGNIVYEKNCRNEAGLSADPYVYNWTAWSEDSDGENGTGQSHHNVFPDGKPFPHHPGWRRWNFIYVFHTLGQYFQKLGRCSVRVSVNTANVTLGPQLMEVTVYRRHGRAYVPIAQVKDVYVVTDQIPVFVTMFQKNDRNSSDATFLKDLPIMFDVLIHDPSHFLNYSTINYKWSFGDNTGLFVSTNHTVNHTYVLNGTFSLNLTVKAAAPGPCPPPPPPPRPSKPTPSLATTLKSYDSNTPGPAGDNPLELSRIPDENCQINRYGHFQATITIVEGILEVNIIQMTDVLMPVPWPESSLIDFVVTCQGSIPTEVCTIISDPTCEITQNTVCSPVDVDEMCLLTVRRTFNGSGTYCVNLTLGDDTSLALTSTLISVPDRDPASPLRMANEFDYKDDDDKLEHHHHHH

SEQ ID NO: 256 - DNA, 1551 bp, Artificial Sequence
  source 1..1551: mol_type = other DNA
atggaatgtctctactatttcctgggatttctgctcctggctgcaagattgccacttgatgccgccaaacgatttcatgatgtgctgggcaatgaaagaccttctgcttacatgagggagcacaatcaattaaatggctggtcttctgatgaaaatgactggaatgaaaaactctacccagtgtggaagcggggagacatgaggtggaaaaactcctggaagggaggccgtgtgcaggcggtcctgaccagtgactcaccagccctcgtgggctcaaatataacatttgcggtgaacctgatattccctagatgccaaaaggaagatgccaatggcaacatagtctatgagaagaactgcagaaatgaggctggtttatctgctgatccgtatgtttacaactggacagcatggtcagaggacagtgacggggaaaatggcaccggccaaagccatcataacgtcttccctgatgggaaaccttttcctcaccaccccggatggagaagatggaatttcatctacgtcttccacacacttggtcagtatttccagaaattgggacgatgttcagtgagagtttctgtgaacacagccaatgtgacacttgggcctcaactcatggaagtgactgtctacagaagacatggacgggcatatgttcccatcgcacaagtgaaagatgtgtacgtggtaacagatcagattcctgtgtttgtgactatgttccagaagaacgatcgaaattcatccgacgcaaccttcctcaaagatctccccattatgtttgatgtcctgattcatgatcctagccacttcctcaattattctaccattaactacaagtggagcttcggggataatactggcctgtttgtttccaccaatcatactgtgaatcacacgtatgtgctcaatggaaccttcagccttaacctcactgtgaaagctgcagcaccaggaccttgtccgccaccgccaccaccacccagaccttcaaaacccaccccttctttagcaactactctaaaatcttatgattcaaacaccccaggacctgctggtgacaaccccctggagctgagtaggattcctgatgaaaactgccagattaacagatatggccactttcaagccaccatcacaattgtagagggaatcttagaggttaacatcatccagatgacagacgtcctgatgccggtgccatggcctgaaagctccctaatagactttgtcgtgacctgccaagggagcattcccacggaggtctgtaccatcatttctgaccccacctgcgagatcacccagaacacagtctgcagccctgtggatgtggatgagatgtgtctgctgactgtgagacgaaccttcaatgggtctgggacgtactgtgtgaacctcaccctgggggatgacacaagcctggctctcacgagcaccctgatttctgttcctgacagagacccagcctcgcctttaaggatggcaaacgaattcgattataaggatgacgatgacaagctcgagcatcaccaccatcaccactaa

SEQ ID NO: 257 - protein, 516 aa, Artificial Sequence
MECLYYFLGFLLLAARLPLDAAKRFHDVLGNERPSAYMREHNQLNGWSSDENDWNEKLYPVWKRGDMRWKNSWKGGRVQAVLTSDSPALVGSNITFAVNLIFPRCQKEDANGNIVYEKNCRNEAGLSADPYVYNWTAWSEDSDGENGTGQSHHNVFPDGKPFPHHPGWRRWNFIYVFHTLGQYFQKLGRCSVRVSVNTANVTLGPQLMEVTVYRRHGRAYVPIAQVKDVYVVTDQIPVFVTMFQKNDRNSSDETFLKDLPIMFAVLIHDPSHFLNYSTINYKWSFGDNTGLFVSTNHTVNHTYVLNGTFSLNLTVKAAAPGPCPPPPPPPRPSKPTPSLATTLKSYDSNTPGPAGDNPLELSRIPDENCQINRYGHFQATITIVEGILEVNIIQMTDVLMPVPWPESSLIDFVVTCQGSIPTEVCTIISDPTCEITQNTVCSPVDVDEMCLLTVRRTFNGSGTYCVNLTLGDDTSLALTSTLISVPDRDPASPLRMANEFDYKDDDDKLEHHHHHH

SEQ ID NO: 258 - DNA, 1551 bp, Artificial Sequence
  source 1..1551: mol_type = other DNA
atggaatgtctctactatttcctgggatttctgctcctggctgcaagattgccacttgatgccgccaaacgatttcatgatgtgctgggcaatgaaagaccttctgcttacatgagggagcacaatcaattaaatggctggtcttctgatgaaaatgactggaatgaaaaactctacccagtgtggaagcggggagacatgaggtggaaaaactcctggaagggaggccgtgtgcaggcggtcctgaccagtgactcaccagccctcgtgggctcaaatataacatttgcggtgaacctgatattccctagatgccaaaaggaagatgccaatggcaacatagtctatgagaagaactgcagaaatgaggctggtttatctgctgatccgtatgtttacaactggacagcatggtcagaggacagtgacggggaaaatggcaccggccaaagccatcataacgtcttccctgatgggaaaccttttcctcaccaccccggatggagaagatggaatttcatctacgtcttccacacacttggtcagtatttccagaaattgggacgatgttcagtgagagtttctgtgaacacagccaatgtgacacttgggcctcaactcatggaagtgactgtctacagaagacatggacgggcatatgttcccatcgcacaagtgaaagatgtgtacgtggtaacagatcagattcctgtgtttgtgactatgttccagaagaacgatcgaaattcatccgacgaaaccttcctcaaagatctccccattatgtttgctgtcctgattcatgatcctagccacttcctcaattattctaccattaactacaagtggagcttcggggataatactggcctgtttgtttccaccaatcatactgtgaatcacacgtatgtgctcaatggaaccttcagccttaacctcactgtgaaagctgcagcaccaggaccttgtccgccaccgccaccaccacccagaccttcaaaacccaccccttctttagcaactactctaaaatcttatgattcaaacaccccaggacctgctggtgacaaccccctggagctgagtaggattcctgatgaaaactgccagattaacagatatggccactttcaagccaccatcacaattgtagagggaatcttagaggttaacatcatccagatgacagacgtcctgatgccggtgccatggcctgaaagctccctaatagactttgtcgtgacctgccaagggagcattcccacggaggtctgtaccatcatttctgaccccacctgcgagatcacccagaacacagtctgcagccctgtggatgtggatgagatgtgtctgctgactgtgagacgaaccttcaatgggtctgggacgtactgtgtgaacctcaccctgggggatgacacaagcctggctctcacgagcaccctgatttctgttcctgacagagacccagcctcgcctttaaggatggcaaacgaattcgattataaggatgacgatgacaagctcgagcatcaccaccatcaccactaa

SEQ ID NO: 259 - protein, 516 aa, Artificial Sequence
MECLYYFLGFLLLAARLPLDAAKRFHDVLGNERPSAYMREHNQLNGWSSDENDWNEKLYPVWKRGDMRWKNSWKGGRVQAVLTSDSPALVGSNITFAVNLIFPRCQKEDANGNIVYEKNCRNEAGLSADPYVYNWTAWSEDSDGENGTGQSHHNVFPDGKPFPHHPGWRRWNFIYVFHTLGQYFQKLGRCSVRVSVNTANVTLGPQLMEVTVYRRHGRAYVPIAQVKDVYVVTDQIPVFVTMFQKNDRNSSDETFLKDLPIMFDVLIHDPSAFLNYSTINYKWSFGDNTGLFVSTNHTVNHTYVLNGTFSLNLTVKAAAPGPCPPPPPPPRPSKPTPSLATTLKSYDSNTPGPAGDNPLELSRIPDENCQINRYGHFQATITIVEGILEVNIIQMTDVLMPVPWPESSLIDFVVTCQGSIPTEVCTIISDPTCEITQNTVCSPVDVDEMCLLTVRRTFNGSGTYCVNLTLGDDTSLALTSTLISVPDRDPASPLRMANEFDYKDDDDKLEHHHHHH

SEQ ID NO: 260 - DNA, 1551 bp, Artificial Sequence
  source 1..1551: mol_type = other DNA
atggaatgtctctactatttcctgggatttctgctcctggctgcaagattgccacttgatgccgccaaacgatttcatgatgtgctgggcaatgaaagaccttctgcttacatgagggagcacaatcaattaaatggctggtcttctgatgaaaatgactggaatgaaaaactctacccagtgtggaagcggggagacatgaggtggaaaaactcctggaagggaggccgtgtgcaggcggtcctgaccagtgactcaccagccctcgtgggctcaaatataacatttgcggtgaacctgatattccctagatgccaaaaggaagatgccaatggcaacatagtctatgagaagaactgcagaaatgaggctggtttatctgctgatccgtatgtttacaactggacagcatggtcagaggacagtgacggggaaaatggcaccggccaaagccatcataacgtcttccctgatgggaaaccttttcctcaccaccccggatggagaagatggaatttcatctacgtcttccacacacttggtcagtatttccagaaattgggacgatgttcagtgagagtttctgtgaacacagccaatgtgacacttgggcctcaactcatggaagtgactgtctacagaagacatggacgggcatatgttcccatcgcacaagtgaaagatgtgtacgtggtaacagatcagattcctgtgtttgtgactatgttccagaagaacgatcgaaattcatccgacgaaaccttcctcaaagatctccccattatgtttgatgtcctgattcatgatcctagcgccttcctcaattattctaccattaactacaagtggagcttcggggataatactggcctgtttgtttccaccaatcatactgtgaatcacacgtatgtgctcaatggaaccttcagccttaacctcactgtgaaagctgcagcaccaggaccttgtccgccaccgccaccaccacccagaccttcaaaacccaccccttctttagcaactactctaaaatcttatgattcaaacaccccaggacctgctggtgacaaccccctggagctgagtaggattcctgatgaaaactgccagattaacagatatggccactttcaagccaccatcacaattgtagagggaatcttagaggttaacatcatccagatgacagacgtcctgatgccggtgccatggcctgaaagctccctaatagactttgtcgtgacctgccaagggagcattcccacggaggtctgtaccatcatttctgaccccacctgcgagatcacccagaacacagtctgcagccctgtggatgtggatgagatgtgtctgctgactgtgagacgaaccttcaatgggtctgggacgtactgtgtgaacctcaccctgggggatgacacaagcctggctctcacgagcaccctgatttctgttcctgacagagacccagcctcgcctttaaggatggcaaacgaattcgattataaggatgacgatgacaagctcgagcatcaccaccatcaccactaa

SEQ ID NO: 261 - protein, 516 aa, Artificial Sequence
MECLYYFLGFLLLAARLPLDAAKRFHDVLGNERPSAYMREHNQLNGWSSDENDWNEKLYPVWKRGDMRWKNSWKGGRVQAVLTSDSPALVGSNITFAVNLIFPRCQKEDANGNIVYEKNCRNEAGLSADPYVYNWTAWSEDSDGENGTGQSHHNVFPDGKPFPHHPGWRRWNFIYVFHTLGQYFQKLGRCSVRVSVNTANVTLGPQLMEVTVYRRHGRAYVPIAQVKDVYVVTDQIPVFVTMFQKNDRNSSDETFLKDLPIMFDVLIHDPSHFLNYSTINYKWSFGDNTGLFVSTNATVNHTYVLNGTFSLNLTVKAAAPGPCPPPPPPPRPSKPTPSLATTLKSYDSNTPGPAGDNPLELSRIPDENCQINRYGHFQATITIVEGILEVNIIQMTDVLMPVPWPESSLIDFVVTCQGSIPTEVCTIISDPTCEITQNTVCSPVDVDEMCLLTVRRTFNGSGTYCVNLTLGDDTSLALTSTLISVPDRDPASPLRMANEFDYKDDDDKLEHHHHHH

SEQ ID NO: 262 - DNA, 1551 bp, Artificial Sequence
  source 1..1551: mol_type = other DNA
atggaatgtctctactatttcctgggatttctgctcctggctgcaagattgccacttgatgccgccaaacgatttcatgatgtgctgggcaatgaaagaccttctgcttacatgagggagcacaatcaattaaatggctggtcttctgatgaaaatgactggaatgaaaaactctacccagtgtggaagcggggagacatgaggtggaaaaactcctggaagggaggccgtgtgcaggcggtcctgaccagtgactcaccagccctcgtgggctcaaatataacatttgcggtgaacctgatattccctagatgccaaaaggaagatgccaatggcaacatagtctatgagaagaactgcagaaatgaggctggtttatctgctgatccgtatgtttacaactggacagcatggtcagaggacagtgacggggaaaatggcaccggccaaagccatcataacgtcttccctgatgggaaaccttttcctcaccaccccggatggagaagatggaatttcatctacgtcttccacacacttggtcagtatttccagaaattgggacgatgttcagtgagagtttctgtgaacacagccaatgtgacacttgggcctcaactcatggaagtgactgtctacagaagacatggacgggcatatgttcccatcgcacaagtgaaagatgtgtacgtggtaacagatcagattcctgtgtttgtgactatgttccagaagaacgatcgaaattcatccgacgaaaccttcctcaaagatctccccattatgtttgatgtcctgattcatgatcctagccacttcctcaattattctaccattaactacaagtggagcttcggggataatactggcctgtttgtttccaccaatgctactgtgaatcacacgtatgtgctcaatggaaccttcagccttaacctcactgtgaaagctgcagcaccaggaccttgtccgccaccgccaccaccacccagaccttcaaaacccaccccttctttagcaactactctaaaatcttatgattcaaacaccccaggacctgctggtgacaaccccctggagctgagtaggattcctgatgaaaactgccagattaacagatatggccactttcaagccaccatcacaattgtagagggaatcttagaggttaacatcatccagatgacagacgtcctgatgccggtgccatggcctgaaagctccctaatagactttgtcgtgacctgccaagggagcattcccacggaggtctgtaccatcatttctgaccccacctgcgagatcacccagaacacagtctgcagccctgtggatgtggatgagatgtgtctgctgactgtgagacgaaccttcaatgggtctgggacgtactgtgtgaacctcaccctgggggatgacacaagcctggctctcacgagcaccctgatttctgttcctgacagagacccagcctcgcctttaaggatggcaaacgaattcgattataaggatgacgatgacaagctcgagcatcaccaccatcaccactaa

SEQ ID NO: 263 - protein, 516 aa, Artificial Sequence
MECLYYFLGFLLLAARLPLDAAKRFHDVLGNERPSAYMREHNQLNGWSSDENDWNEKLYPVWKRGDMRWKNSWKGGRVQAVLTSDSPALVGSNITFAVNLIFPRCQKEDANGNIVYEKNCRNEAGLSADPYVYNWTAWSEDSDGENGTGQSHHNVFPDGKPFPHHPGWRRWNFIYVFHTLGQYFQKLGRCSVRVSVNTANVTLGPQLMEVTVYRRHGRAYVPIAQVKDVYVVTDQIPVFVTMFQKNDRNSSDETFLKDLPIMFDVLIHDPSHFLNYSTINYKWSFGDNTGLFVSTNHTVNHTYVLNGTFSLNLTVKAAAPGPCPPPPPPPRPSKPTPSLATTLKSYDSNTPGPAGDNPLELSRIPDENCQINRYGAFQATITIVEGILEVNIIQMTDVLMPVPWPESSLIDFVVTCQGSIPTEVCTIISDPTCEITQNTVCSPVDVDEMCLLTVRRTFNGSGTYCVNLTLGDDTSLALTSTLISVPDRDPASPLRMANEFDYKDDDDKLEHHHHHH

SEQ ID NO: 264 - DNA, 1551 bp, Artificial Sequence
  source 1..1551: mol_type = other DNA
atggaatgtctctactatttcctgggatttctgctcctggctgcaagattgccacttgatgccgccaaacgatttcatgatgtgctgggcaatgaaagaccttctgcttacatgagggagcacaatcaattaaatggctggtcttctgatgaaaatgactggaatgaaaaactctacccagtgtggaagcggggagacatgaggtggaaaaactcctggaagggaggccgtgtgcaggcggtcctgaccagtgactcaccagccctcgtgggctcaaatataacatttgcggtgaacctgatattccctagatgccaaaaggaagatgccaatggcaacatagtctatgagaagaactgcagaaatgaggctggtttatctgctgatccgtatgtttacaactggacagcatggtcagaggacagtgacggggaaaatggcaccggccaaagccatcataacgtcttccctgatgggaaaccttttcctcaccaccccggatggagaagatggaatttcatctacgtcttccacacacttggtcagtatttccagaaattgggacgatgttcagtgagagtttctgtgaacacagccaatgtgacacttgggcctcaactcatggaagtgactgtctacagaagacatggacgggcatatgttcccatcgcacaagtgaaagatgtgtacgtggtaacagatcagattcctgtgtttgtgactatgttccagaagaacgatcgaaattcatccgacgaaaccttcctcaaagatctccccattatgtttgatgtcctgattcatgatcctagccacttcctcaattattctaccattaactacaagtggagcttcggggataatactggcctgtttgtttccaccaatcatactgtgaatcacacgtatgtgctcaatggaaccttcagccttaacctcactgtgaaagctgcagcaccaggaccttgtccgccaccgccaccaccacccagaccttcaaaacccaccccttctttagcaactactctaaaatcttatgattcaaacaccccaggacctgctggtgacaaccccctggagctgagtaggattcctgatgaaaactgccagattaacagatatggcgcctttcaagccaccatcacaattgtagagggaatcttagaggttaacatcatccagatgacagacgtcctgatgccggtgccatggcctgaaagctccctaatagactttgtcgtgacctgccaagggagcattcccacggaggtctgtaccatcatttctgaccccacctgcgagatcacccagaacacagtctgcagccctgtggatgtggatgagatgtgtctgctgactgtgagacgaaccttcaatgggtctgggacgtactgtgtgaacctcaccctgggggatgacacaagcctggctctcacgagcaccctgatttctgttcctgacagagacccagcctcgcctttaaggatggcaaacgaattcgattataaggatgacgatgacaagctcgagcatcaccaccatcaccactaa

SEQ ID NO: 265 - protein, 516 aa, Artificial Sequence
MECLYYFLGFLLLAARLPLDAAKRFHDVLGNERPSAYMREHNQLNGWSSDENDWNEKLYPVWKRGDMRWKNSWKGGRVQAVLTSDSPALVGSNITFAVNLIFPRCQKEDANGNIVYEKNCRNEAGLSADPYVYNWTAWSEDSDGENGTGQSHHNVFPDGKPFPHHPGWRRWNFIYVFHTLGQYFQKLGRCSVRVSVNTANVTLGPQLMEVTVYRRHGRAYVPIAQVKDVYVVTDQIPVFVTMFQKNAANSSDETFLKDLPIMFDVLIHDPSHFLNYSTINYKWSFGDNTGLFVSTNHTVNHTYVLNGTFSLNLTVKAAAPGPCPPPPPPPRPSKPTPSLATTLKSYDSNTPGPAGDNPLELSRIPDENCQINRYGHFQATITIVEGILEVNIIQMTDVLMPVPWPESSLIDFVVTCQGSIPTEVCTIISDPTCEITQNTVCSPVDVDEMCLLTVRRTFNGSGTYCVNLTLGDDTSLALTSTLISVPDRDPASPLRMANEFDYKDDDDKLEHHHHHH

SEQ ID NO: 266 - DNA, 1551 bp, Artificial Sequence
  source 1..1551: mol_type = other DNA
atggaatgtctctactatttcctgggatttctgctcctggctgcaagattgccacttgatgccgccaaacgatttcatgatgtgctgggcaatgaaagaccttctgcttacatgagggagcacaatcaattaaatggctggtcttctgatgaaaatgactggaatgaaaaactctacccagtgtggaagcggggagacatgaggtggaaaaactcctggaagggaggccgtgtgcaggcggtcctgaccagtgactcaccagccctcgtgggctcaaatataacatttgcggtgaacctgatattccctagatgccaaaaggaagatgccaatggcaacatagtctatgagaagaactgcagaaatgaggctggtttatctgctgatccgtatgtttacaactggacagcatggtcagaggacagtgacggggaaaatggcaccggccaaagccatcataacgtcttccctgatgggaaaccttttcctcaccaccccggatggagaagatggaatttcatctacgtcttccacacacttggtcagtatttccagaaattgggacgatgttcagtgagagtttctgtgaacacagccaatgtgacacttgggcctcaactcatggaagtgactgtctacagaagacatggacgggcatatgttcccatcgcacaagtgaaagatgtgtacgtggtaacagatcagattcctgtgtttgtgactatgttccagaagaacgctgcaaattcatccgacgaaaccttcctcaaagatctccccattatgtttgatgtcctgattcatgatcctagccacttcctcaattattctaccattaactacaagtggagcttcggggataatactggcctgtttgtttccaccaatcatactgtgaatcacacgtatgtgctcaatggaaccttcagccttaacctcactgtgaaagctgcagcaccaggaccttgtccgccaccgccaccaccacccagaccttcaaaacccaccccttctttagcaactactctaaaatcttatgattcaaacaccccaggacctgctggtgacaaccccctggagctgagtaggattcctgatgaaaactgccagattaacagatatggccactttcaagccaccatcacaattgtagagggaatcttagaggttaacatcatccagatgacagacgtcctgatgccggtgccatggcctgaaagctccctaatagactttgtcgtgacctgccaagggagcattcccacggaggtctgtaccatcatttctgaccccacctgcgagatcacccagaacacagtctgcagccctgtggatgtggatgagatgtgtctgctgactgtgagacgaaccttcaatgggtctgggacgtactgtgtgaacctcaccctgggggatgacacaagcctggctctcacgagcaccctgatttctgttcctgacagagacccagcctcgcctttaaggatggcaaacgaattcgattataaggatgacgatgacaagctcgagcatcaccaccatcaccactaa

SEQ ID NO: 267 - protein, 516 aa, Artificial Sequence
MECLYYFLGFLLLAARLPLDAAKRFHDVLGNERPSAYMREHNQLNGWSSDENDWNEKLYPVWKRGDMRWKNSWKGGRVQAVLTSDSPALVGSNITFAVNLIFPRCQKEDANGNIVYEKNCRNEAGLSADPYVYNWTAWSEDSDGENGTGQSHHNVFPDGKPFPHHPGWRRWNFIYVFHTLGQYFQKLGRCSVRVSVNTANVTLGPQLMEVTVYRRHGRAYVPIAQVKDVYVVTDQIPVFVTMFQKNDRNSSDETFLKDLPIMFDVLIHDPSHFLNYSTINYKWSFGANTGLFVSTNHTVNHTYVLNGTFSLNLTVKAAAPGPCPPPPPPPRPSKPTPSLATTLKSYDSNTPGPAGDNPLELSRIPDENCQINRYGHFQATITIVEGILEVNIIQMTDVLMPVPWPESSLIDFVVTCQGSIPTEVCTIISDPTCEITQNTVCSPVDVDEMCLLTVRRTFNGSGTYCVNLTLGDDTSLALTSTLISVPDRDPASPLRMANEFDYKDDDDKLEHHHHHH

SEQ ID NO: 268 - DNA, 1551 bp, Artificial Sequence
  source 1..1551: mol_type = other DNA
atggaatgtctctactatttcctgggatttctgctcctggctgcaagattgccacttgatgccgccaaacgatttcatgatgtgctgggcaatgaaagaccttctgcttacatgagggagcacaatcaattaaatggctggtcttctgatgaaaatgactggaatgaaaaactctacccagtgtggaagcggggagacatgaggtggaaaaactcctggaagggaggccgtgtgcaggcggtcctgaccagtgactcaccagccctcgtgggctcaaatataacatttgcggtgaacctgatattccctagatgccaaaaggaagatgccaatggcaacatagtctatgagaagaactgcagaaatgaggctggtttatctgctgatccgtatgtttacaactggacagcatggtcagaggacagtgacggggaaaatggcaccggccaaagccatcataacgtcttccctgatgggaaaccttttcctcaccaccccggatggagaagatggaatttcatctacgtcttccacacacttggtcagtatttccagaaattgggacgatgttcagtgagagtttctgtgaacacagccaatgtgacacttgggcctcaactcatggaagtgactgtctacagaagacatggacgggcatatgttcccatcgcacaagtgaaagatgtgtacgtggtaacagatcagattcctgtgtttgtgactatgttccagaagaacgatcgaaattcatccgacgaaaccttcctcaaagatctccccattatgtttgatgtcctgattcatgatcctagccacttcctcaattattctaccattaactacaagtggagcttcggggctaatactggcctgtttgtttccaccaatcatactgtgaatcacacgtatgtgctcaatggaaccttcagccttaacctcactgtgaaagctgcagcaccaggaccttgtccgccaccgccaccaccacccagaccttcaaaacccaccccttctttagcaactactctaaaatcttatgattcaaacaccccaggacctgctggtgacaaccccctggagctgagtaggattcctgatgaaaactgccagattaacagatatggccactttcaagccaccatcacaattgtagagggaatcttagaggttaacatcatccagatgacagacgtcctgatgccggtgccatggcctgaaagctccctaatagactttgtcgtgacctgccaagggagcattcccacggaggtctgtaccatcatttctgaccccacctgcgagatcacccagaacacagtctgcagccctgtggatgtggatgagatgtgtctgctgactgtgagacgaaccttcaatgggtctgggacgtactgtgtgaacctcaccctgggggatgacacaagcctggctctcacgagcaccctgatttctgttcctgacagagacccagcctcgcctttaaggatggcaaacgaattcgattataaggatgacgatgacaagctcgagcatcaccaccatcaccactaa

SEQ ID NO: 269 - protein, 516 aa, Artificial Sequence
MECLYYFLGFLLLAARLPLDAAKRFHDVLGNERPSAYMREHNQLNGWSSDENDWNEKLYPVWKRGDMRWKNSWKGGRVQAVLTSDSPALVGSNITFAVNLIFPRCQKEDANGNIVYEKNCRNEAGLSADPYVYNWTAWSEDSDGENGTGQSHHNVFPDGKPFPHHPGWRRWNFIYVFHTLGQYFQKLGRCSVRVSVNTANVTLGPQLMEVTVYRRHGRAYVPIAQVKDVYVVTDQIPVFVTMFQKNDRNSSDETFLKDLPIMFDVLIHDPSHFLNYSTINYKWSFGDNTGLFVSTNHTVNATYVLNGTFSLNLTVKAAAPGPCPPPPPPPRPSKPTPSLATTLKSYDSNTPGPAGDNPLELSRIPDENCQINRYGHFQATITIVEGILEVNIIQMTDVLMPVPWPESSLIDFVVTCQGSIPTEVCTIISDPTCEITQNTVCSPVDVDEMCLLTVRRTFNGSGTYCVNLTLGDDTSLALTSTLISVPDRDPASPLRMANEFDYKDDDDKLEHHHHHH

SEQ ID NO: 270 - DNA, 1551 bp, Artificial Sequence
  source 1..1551: mol_type = other DNA
atggaatgtctctactatttcctgggatttctgctcctggctgcaagattgccacttgatgccgccaaacgatttcatgatgtgctgggcaatgaaagaccttctgcttacatgagggagcacaatcaattaaatggctggtcttctgatgaaaatgactggaatgaaaaactctacccagtgtggaagcggggagacatgaggtggaaaaactcctggaagggaggccgtgtgcaggcggtcctgaccagtgactcaccagccctcgtgggctcaaatataacatttgcggtgaacctgatattccctagatgccaaaaggaagatgccaatggcaacatagtctatgagaagaactgcagaaatgaggctggtttatctgctgatccgtatgtttacaactggacagcatggtcagaggacagtgacggggaaaatggcaccggccaaagccatcataacgtcttccctgatgggaaaccttttcctcaccaccccggatggagaagatggaatttcatctacgtcttccacacacttggtcagtatttccagaaattgggacgatgttcagtgagagtttctgtgaacacagccaatgtgacacttgggcctcaactcatggaagtgactgtctacagaagacatggacgggcatatgttcccatcgcacaagtgaaagatgtgtacgtggtaacagatcagattcctgtgtttgtgactatgttccagaagaacgatcgaaattcatccgacgaaaccttcctcaaagatctccccattatgtttgatgtcctgattcatgatcctagccacttcctcaattattctaccattaactacaagtggagcttcggggataatactggcctgtttgtttccaccaatcatactgtgaatgccacgtatgtgctcaatggaaccttcagccttaacctcactgtgaaagctgcagcaccaggaccttgtccgccaccgccaccaccacccagaccttcaaaacccaccccttctttagcaactactctaaaatcttatgattcaaacaccccaggacctgctggtgacaaccccctggagctgagtaggattcctgatgaaaactgccagattaacagatatggccactttcaagccaccatcacaattgtagagggaatcttagaggttaacatcatccagatgacagacgtcctgatgccggtgccatggcctgaaagctccctaatagactttgtcgtgacctgccaagggagcattcccacggaggtctgtaccatcatttctgaccccacctgcgagatcacccagaacacagtctgcagccctgtggatgtggatgagatgtgtctgctgactgtgagacgaaccttcaatgggtctgggacgtactgtgtgaacctcaccctgggggatgacacaagcctggctctcacgagcaccctgatttctgttcctgacagagacccagcctcgcctttaaggatggcaaacgaattcgattataaggatgacgatgacaagctcgagcatcaccaccatcaccactaa

SEQ ID NO: 271 - protein, 516 aa, Artificial Sequence
MECLYYFLGFLLLAARLPLDAAKRFHDVLGNERPSAYMREHNQLNGWSSDENDWNEKLYPVWKRGDMRWKNSWKGGRVQAVLTSDSPALVGSNITFAVNLIFPRCQKEDANGNIVYEKNCRNEAGLSADPYVYNWTAWSEDSDGENGTGQSHHNVFPDGKPFPHHPGWRRWNFIYVFHTLGQYFQKLGRCSVRVSVNTANVTLGPQLMEVTVYRRHGRAYVPIAQVKDVYVVTDQIPVFVTMFQKNDRNSSDETFLKDLPIMFDVLIHDPSHFLNYSTINYKWSFGDNTGLFVSTNHTVNHTYVLNGTFSLNLTVKAAAPGPCPPPPPPPAPSAPTPSLATTLKSYDSNTPGPAGDNPLELSRIPDENCQINRYGHFQATITIVEGILEVNIIQMTDVLMPVPWPESSLIDFVVTCQGSIPTEVCTIISDPTCEITQNTVCSPVDVDEMCLLTVRRTFNGSGTYCVNLTLGDDTSLALTSTLISVPDRDPASPLRMANEFDYKDDDDKLEHHHHHH

SEQ ID NO: 272 - DNA, 1551 bp, Artificial Sequence
  source 1..1551: mol_type = other DNA
atggaatgtctctactatttcctgggatttctgctcctggctgcaagattgccacttgatgccgccaaacgatttcatgatgtgctgggcaatgaaagaccttctgcttacatgagggagcacaatcaattaaatggctggtcttctgatgaaaatgactggaatgaaaaactctacccagtgtggaagcggggagacatgaggtggaaaaactcctggaagggaggccgtgtgcaggcggtcctgaccagtgactcaccagccctcgtgggctcaaatataacatttgcggtgaacctgatattccctagatgccaaaaggaagatgccaatggcaacatagtctatgagaagaactgcagaaatgaggctggtttatctgctgatccgtatgtttacaactggacagcatggtcagaggacagtgacggggaaaatggcaccggccaaagccatcataacgtcttccctgatgggaaaccttttcctcaccaccccggatggagaagatggaatttcatctacgtcttccacacacttggtcagtatttccagaaattgggacgatgttcagtgagagtttctgtgaacacagccaatgtgacacttgggcctcaactcatggaagtgactgtctacagaagacatggacgggcatatgttcccatcgcacaagtgaaagatgtgtacgtggtaacagatcagattcctgtgtttgtgactatgttccagaagaacgatcgaaattcatccgacgaaaccttcctcaaagatctccccattatgtttgatgtcctgattcatgatcctagccacttcctcaattattctaccattaactacaagtggagcttcggggataatactggcctgtttgtttccaccaatcatactgtgaatcacacgtatgtgctcaatggaaccttcagccttaacctcactgtgaaagctgcagcaccaggaccttgtccgccaccgccaccaccacccgcaccttcagcacccaccccttctttagcaactactctaaaatcttatgattcaaacaccccaggacctgctggtgacaaccccctggagctgagtaggattcctgatgaaaactgccagattaacagatatggccactttcaagccaccatcacaattgtagagggaatcttagaggttaacatcatccagatgacagacgtcctgatgccggtgccatggcctgaaagctccctaatagactttgtcgtgacctgccaagggagcattcccacggaggtctgtaccatcatttctgaccccacctgcgagatcacccagaacacagtctgcagccctgtggatgtggatgagatgtgtctgctgactgtgagacgaaccttcaatgggtctgggacgtactgtgtgaacctcaccctgggggatgacacaagcctggctctcacgagcaccctgatttctgttcctgacagagacccagcctcgcctttaaggatggcaaacgaattcgattataaggatgacgatgacaagctcgagcatcaccaccatcaccactaa

SEQ ID NO: 273 - protein, 516 aa, Artificial Sequence
MECLYYFLGFLLLAARLPLDAAKRFHDVLGNERPSAYMREHNQLNGWSSDENDWNEKLYPVWKRGDMRWKNSWKGGRVQAVLTSDSPALVGSNITFAVNLIFPRCQKEDANGNIVYEKNCRNEAGLSADPYVYNWTAWSEDSDGENGTGQSHHNVFPDGKPFPHHPGWRRWNFIYVFHTLGQYFQKLGRCSVRVSVNTANVTLGPQLMEVTVYRRHGRAYVPIAQVKDVYVVTDQIPVFVTMFQKNDRNSSDETFLKDLPIMFDVLIHDPSHFLNYSTINYKWSFGDNTGLFVSTNHTVNHTYVLNGTFSLNLTVKAAAPGPCPPPPPPPRPSKPTPSLATTLASYASNTPGPAGDNPLELSRIPDENCQINRYGHFQATITIVEGILEVNIIQMTDVLMPVPWPESSLIDFVVTCQGSIPTEVCTIISDPTCEITQNTVCSPVDVDEMCLLTVRRTFNGSGTYCVNLTLGDDTSLALTSTLISVPDRDPASPLRMANEFDYKDDDDKLEHHHHHH

SEQ ID NO: 274 - DNA, 1551 bp, Artificial Sequence
  source 1..1551: mol_type = other DNA
atggaatgtctctactatttcctgggatttctgctcctggctgcaagattgccacttgatgccgccaaacgatttcatgatgtgctgggcaatgaaagaccttctgcttacatgagggagcacaatcaattaaatggctggtcttctgatgaaaatgactggaatgaaaaactctacccagtgtggaagcggggagacatgaggtggaaaaactcctggaagggaggccgtgtgcaggcggtcctgaccagtgactcaccagccctcgtgggctcaaatataacatttgcggtgaacctgatattccctagatgccaaaaggaagatgccaatggcaacatagtctatgagaagaactgcagaaatgaggctggtttatctgctgatccgtatgtttacaactggacagcatggtcagaggacagtgacggggaaaatggcaccggccaaagccatcataacgtcttccctgatgggaaaccttttcctcaccaccccggatggagaagatggaatttcatctacgtcttccacacacttggtcagtatttccagaaattgggacgatgttcagtgagagtttctgtgaacacagccaatgtgacacttgggcctcaactcatggaagtgactgtctacagaagacatggacgggcatatgttcccatcgcacaagtgaaagatgtgtacgtggtaacagatcagattcctgtgtttgtgactatgttccagaagaacgatcgaaattcatccgacgaaaccttcctcaaagatctccccattatgtttgatgtcctgattcatgatcctagccacttcctcaattattctaccattaactacaagtggagcttcggggataatactggcctgtttgtttccaccaatcatactgtgaatcacacgtatgtgctcaatggaaccttcagccttaacctcactgtgaaagctgcagcaccaggaccttgtccgccaccgccaccaccacccagaccttcaaaacccaccccttctttagcaactactctagcatcttatgcttcaaacaccccaggacctgctggtgacaaccccctggagctgagtaggattcctgatgaaaactgccagattaacagatatggccactttcaagccaccatcacaattgtagagggaatcttagaggttaacatcatccagatgacagacgtcctgatgccggtgccatggcctgaaagctccctaatagactttgtcgtgacctgccaagggagcattcccacggaggtctgtaccatcatttctgaccccacctgcgagatcacccagaacacagtctgcagccctgtggatgtggatgagatgtgtctgctgactgtgagacgaaccttcaatgggtctgggacgtactgtgtgaacctcaccctgggggatgacacaagcctggctctcacgagcaccctgatttctgttcctgacagagacccagcctcgcctttaaggatggcaaacgaattcgattataaggatgacgatgacaagctcgagcatcaccaccatcaccactaa

SEQ ID NO: 275 - protein, 516 aa, Artificial Sequence
MECLYYFLGFLLLAARLPLDAAKRFHDVLGNERPSAYMREHNQLNGWSSDENDWNEKLYPVWKRGDMRWKNSWKGGRVQAVLTSDSPALVGSNITFAVNLIFPRCQKEDANGNIVYEKNCRNEAGLSADPYVYNWTAWSEDSDGENGTGQSHHNVFPDGKPFPHHPGWRRWNFIYVFHTLGQYFQKLGRCSVRVSVNTANVTLGPQLMEVTVYRRHGRAYVPIAQVKDVYVVTDQIPVFVTMFQKNDRNSSDETFLKDLPIMFDVLIHDPSHFLNYSTINYKWSFGDNTGLFVSTNHTVNHTYVLNGTFSLNLTVKAAAPGPCPPPPPPPRPSKPTPSLATTLKSYDSNTPGPAGANPLELSRIPDENCQINRYGHFQATITIVEGILEVNIIQMTDVLMPVPWPESSLIDFVVTCQGSIPTEVCTIISDPTCEITQNTVCSPVDVDEMCLLTVRRTFNGSGTYCVNLTLGDDTSLALTSTLISVPDRDPASPLRMANEFDYKDDDDKLEHHHHHH

SEQ ID NO: 276 - DNA, 1551 bp, Artificial Sequence
  source 1..1551: mol_type = other DNA
atggaatgtctctactatttcctgggatttctgctcctggctgcaagattgccacttgatgccgccaaacgatttcatgatgtgctgggcaatgaaagaccttctgcttacatgagggagcacaatcaattaaatggctggtcttctgatgaaaatgactggaatgaaaaactctacccagtgtggaagcggggagacatgaggtggaaaaactcctggaagggaggccgtgtgcaggcggtcctgaccagtgactcaccagccctcgtgggctcaaatataacatttgcggtgaacctgatattccctagatgccaaaaggaagatgccaatggcaacatagtctatgagaagaactgcagaaatgaggctggtttatctgctgatccgtatgtttacaactggacagcatggtcagaggacagtgacggggaaaatggcaccggccaaagccatcataacgtcttccctgatgggaaaccttttcctcaccaccccggatggagaagatggaatttcatctacgtcttccacacacttggtcagtatttccagaaattgggacgatgttcagtgagagtttctgtgaacacagccaatgtgacacttgggcctcaactcatggaagtgactgtctacagaagacatggacgggcatatgttcccatcgcacaagtgaaagatgtgtacgtggtaacagatcagattcctgtgtttgtgactatgttccagaagaacgatcgaaattcatccgacgaaaccttcctcaaagatctccccattatgtttgatgtcctgattcatgatcctagccacttcctcaattattctaccattaactacaagtggagcttcggggataatactggcctgtttgtttccaccaatcatactgtgaatcacacgtatgtgctcaatggaaccttcagccttaacctcactgtgaaagctgcagcaccaggaccttgtccgccaccgccaccaccacccagaccttcaaaacccaccccttctttagcaactactctaaaatcttatgattcaaacaccccaggacctgctggtgccaaccccctggagctgagtaggattcctgatgaaaactgccagattaacagatatggccactttcaagccaccatcacaattgtagagggaatcttagaggttaacatcatccagatgacagacgtcctgatgccggtgccatggcctgaaagctccctaatagactttgtcgtgacctgccaagggagcattcccacggaggtctgtaccatcatttctgaccccacctgcgagatcacccagaacacagtctgcagccctgtggatgtggatgagatgtgtctgctgactgtgagacgaaccttcaatgggtctgggacgtactgtgtgaacctcaccctgggggatgacacaagcctggctctcacgagcaccctgatttctgttcctgacagagacccagcctcgcctttaaggatggcaaacgaattcgattataaggatgacgatgacaagctcgagcatcaccaccatcaccactaa

SEQ ID NO: 277 - protein, 516 aa, Artificial Sequence
MECLYYFLGFLLLAARLPLDAAKRFHDVLGNERPSAYMREHNQLNGWSSDENDWNEKLYPVWKRGDMRWKNSWKGGRVQAVLTSDSPALVGSNITFAVNLIFPRCQKEDANGNIVYEKNCRNEAGLSADPYVYNWTAWSEDSDGENGTGQSHHNVFPDGKPFPHHPGWRRWNFIYVFHTLGQYFQKLGRCSVRVSVNTANVTLGPQLMEVTVYRRHGRAYVPIAQVKDVYVVTDQIPVFVTMFQKNDRNSSDETFLKDLPIMFDVLIHDPSHFLNYSTINYKWSFGDNTGLFVSTNHTVNHTYVLNGTFSLNLTVKAAAPGPCPPPPPPPRPSKPTPSLATTLKSYDSNTPGPAGDNPLALSRIPDENCQINRYGHFQATITIVEGILEVNIIQMTDVLMPVPWPESSLIDFVVTCQGSIPTEVCTIISDPTCEITQNTVCSPVDVDEMCLLTVRRTFNGSGTYCVNLTLGDDTSLALTSTLISVPDRDPASPLRMANEFDYKDDDDKLEHHHHHH

SEQ ID NO: 278 - DNA, 1551 bp, Artificial Sequence
  source 1..1551: mol_type = other DNA
atggaatgtctctactatttcctgggatttctgctcctggctgcaagattgccacttgatgccgccaaacgatttcatgatgtgctgggcaatgaaagaccttctgcttacatgagggagcacaatcaattaaatggctggtcttctgatgaaaatgactggaatgaaaaactctacccagtgtggaagcggggagacatgaggtggaaaaactcctggaagggaggccgtgtgcaggcggtcctgaccagtgactcaccagccctcgtgggctcaaatataacatttgcggtgaacctgatattccctagatgccaaaaggaagatgccaatggcaacatagtctatgagaagaactgcagaaatgaggctggtttatctgctgatccgtatgtttacaactggacagcatggtcagaggacagtgacggggaaaatggcaccggccaaagccatcataacgtcttccctgatgggaaaccttttcctcaccaccccggatggagaagatggaatttcatctacgtcttccacacacttggtcagtatttccagaaattgggacgatgttcagtgagagtttctgtgaacacagccaatgtgacacttgggcctcaactcatggaagtgactgtctacagaagacatggacgggcatatgttcccatcgcacaagtgaaagatgtgtacgtggtaacagatcagattcctgtgtttgtgactatgttccagaagaacgatcgaaattcatccgacgaaaccttcctcaaagatctccccattatgtttgatgtcctgattcatgatcctagccacttcctcaattattctaccattaactacaagtggagcttcggggataatactggcctgtttgtttccaccaatcatactgtgaatcacacgtatgtgctcaatggaaccttcagccttaacctcactgtgaaagctgcagcaccaggaccttgtccgccaccgccaccaccacccagaccttcaaaacccaccccttctttagcaactactctaaaatcttatgattcaaacaccccaggacctgctggtgacaaccccctggcgctgagtaggattcctgatgaaaactgccagattaacagatatggccactttcaagccaccatcacaattgtagagggaatcttagaggttaacatcatccagatgacagacgtcctgatgccggtgccatggcctgaaagctccctaatagactttgtcgtgacctgccaagggagcattcccacggaggtctgtaccatcatttctgaccccacctgcgagatcacccagaacacagtctgcagccctgtggatgtggatgagatgtgtctgctgactgtgagacgaaccttcaatgggtctgggacgtactgtgtgaacctcaccctgggggatgacacaagcctggctctcacgagcaccctgatttctgttcctgacagagacccagcctcgcctttaaggatggcaaacgaattcgattataaggatgacgatgacaagctcgagcatcaccaccatcaccactaa

SEQ ID NO: 279 - protein, 516 aa, Artificial Sequence
MECLYYFLGFLLLAARLPLDAAKRFHDVLGNERPSAYMREHNQLNGWSSDENDWNEKLYPVWKRGDMRWKNSWKGGRVQAVLTSDSPALVGSNITFAVNLIFPRCQKEDANGNIVYEKNCRNEAGLSADPYVYNWTAWSEDSDGENGTGQSHHNVFPDGKPFPHHPGWRRWNFIYVFHTLGQYFQKLGRCSVRVSVNTANVTLGPQLMEVTVYRRHGRAYVPIAQVKDVYVVTDQIPVFVTMFQKNDRNSSDETFLKDLPIMFDVLIHDPSHFLNYSTINYKWSFGDNTGLFVSTNHTVNHTYVLNGTFSLNLTVKAAAPGPCPPPPPPPRPSKPTPSLATTLKSYDSNTPGPAGDNPLELSRIPDANCQINRYGHFQATITIVEGILEVNIIQMTDVLMPVPWPESSLIDFVVTCQGSIPTEVCTIISDPTCEITQNTVCSPVDVDEMCLLTVRRTFNGSGTYCVNLTLGDDTSLALTSTLISVPDRDPASPLRMANEFDYKDDDDKLEHHHHHH

SEQ ID NO: 280 - DNA, 1551 bp, Artificial Sequence
  source 1..1551: mol_type = other DNA
atggaatgtctctactatttcctgggatttctgctcctggctgcaagattgccacttgatgccgccaaacgatttcatgatgtgctgggcaatgaaagaccttctgcttacatgagggagcacaatcaattaaatggctggtcttctgatgaaaatgactggaatgaaaaactctacccagtgtggaagcggggagacatgaggtggaaaaactcctggaagggaggccgtgtgcaggcggtcctgaccagtgactcaccagccctcgtgggctcaaatataacatttgcggtgaacctgatattccctagatgccaaaaggaagatgccaatggcaacatagtctatgagaagaactgcagaaatgaggctggtttatctgctgatccgtatgtttacaactggacagcatggtcagaggacagtgacggggaaaatggcaccggccaaagccatcataacgtcttccctgatgggaaaccttttcctcaccaccccggatggagaagatggaatttcatctacgtcttccacacacttggtcagtatttccagaaattgggacgatgttcagtgagagtttctgtgaacacagccaatgtgacacttgggcctcaactcatggaagtgactgtctacagaagacatggacgggcatatgttcccatcgcacaagtgaaagatgtgtacgtggtaacagatcagattcctgtgtttgtgactatgttccagaagaacgatcgaaattcatccgacgaaaccttcctcaaagatctccccattatgtttgatgtcctgattcatgatcctagccacttcctcaattattctaccattaactacaagtggagcttcggggataatactggcctgtttgtttccaccaatcatactgtgaatcacacgtatgtgctcaatggaaccttcagccttaacctcactgtgaaagctgcagcaccaggaccttgtccgccaccgccaccaccacccagaccttcaaaacccaccccttctttagcaactactctaaaatcttatgattcaaacaccccaggacctgctggtgacaaccccctggagctgagtaggattcctgatgcaaactgccagattaacagatatggccactttcaagccaccatcacaattgtagagggaatcttagaggttaacatcatccagatgacagacgtcctgatgccggtgccatggcctgaaagctccctaatagactttgtcgtgacctgccaagggagcattcccacggaggtctgtaccatcatttctgaccccacctgcgagatcacccagaacacagtctgcagccctgtggatgtggatgagatgtgtctgctgactgtgagacgaaccttcaatgggtctgggacgtactgtgtgaacctcaccctgggggatgacacaagcctggctctcacgagcaccctgatttctgttcctgacagagacccagcctcgcctttaaggatggcaaacgaattcgattataaggatgacgatgacaagctcgagcatcaccaccatcaccactaa

SEQ ID NO: 281 - protein, 516 aa, Artificial Sequence
MECLYYFLGFLLLAARLPLDAAKRFHDVLGNERPSAYMREHNQLNGWSSDENDWNEKLYPVWKRGDMRWKNSWKGGRVQAVLTSDSPALVGSNITFAVNLIFPRCQKEDANGNIVYEKNCRNEAGLSADPYVYNWTAWSEDSDGENGTGQSHHNVFPDGKPFPHHPGWRRWNFIYVFHTLGQYFQKLGRCSVRVSVNTANVTLGPQLMEVTVYRRHGRAYVPIAQVKDVYVVTDQIPVFVTMFQKNDRNSSDETFLKDLPIMFDVLIHDPSHFLNYSTINYKWSFGDNTGLFVSTNHTVNHTYVLNGTFSLNLTVKAAAPGPCPPPPPPPRPSKPTPSLATTLKSYDSNTPGPAGDNPLELSRIPDENCQINAYGHFQATITIVEGILEVNIIQMTDVLMPVPWPESSLIDFVVTCQGSIPTEVCTIISDPTCEITQNTVCSPVDVDEMCLLTVRRTFNGSGTYCVNLTLGDDTSLALTSTLISVPDRDPASPLRMANEFDYKDDDDKLEHHHHHH

SEQ ID NO: 282 - DNA, 1551 bp, Artificial Sequence
  source 1..1551: mol_type = other DNA
atggaatgtctctactatttcctgggatttctgctcctggctgcaagattgccacttgatgccgccaaacgatttcatgatgtgctgggcaatgaaagaccttctgcttacatgagggagcacaatcaattaaatggctggtcttctgatgaaaatgactggaatgaaaaactctacccagtgtggaagcggggagacatgaggtggaaaaactcctggaagggaggccgtgtgcaggcggtcctgaccagtgactcaccagccctcgtgggctcaaatataacatttgcggtgaacctgatattccctagatgccaaaaggaagatgccaatggcaacatagtctatgagaagaactgcagaaatgaggctggtttatctgctgatccgtatgtttacaactggacagcatggtcagaggacagtgacggggaaaatggcaccggccaaagccatcataacgtcttccctgatgggaaaccttttcctcaccaccccggatggagaagatggaatttcatctacgtcttccacacacttggtcagtatttccagaaattgggacgatgttcagtgagagtttctgtgaacacagccaatgtgacacttgggcctcaactcatggaagtgactgtctacagaagacatggacgggcatatgttcccatcgcacaagtgaaagatgtgtacgtggtaacagatcagattcctgtgtttgtgactatgttccagaagaacgatcgaaattcatccgacgaaaccttcctcaaagatctccccattatgtttgatgtcctgattcatgatcctagccacttcctcaattattctaccattaactacaagtggagcttcggggataatactggcctgtttgtttccaccaatcatactgtgaatcacacgtatgtgctcaatggaaccttcagccttaacctcactgtgaaagctgcagcaccaggaccttgtccgccaccgccaccaccacccagaccttcaaaacccaccccttctttagcaactactctaaaatcttatgattcaaacaccccaggacctgctggtgacaaccccctggagctgagtaggattcctgatgaaaactgccagattaacgcatatggccactttcaagccaccatcacaattgtagagggaatcttagaggttaacatcatccagatgacagacgtcctgatgccggtgccatggcctgaaagctccctaatagactttgtcgtgacctgccaagggagcattcccacggaggtctgtaccatcatttctgaccccacctgcgagatcacccagaacacagtctgcagccctgtggatgtggatgagatgtgtctgctgactgtgagacgaaccttcaatgggtctgggacgtactgtgtgaacctcaccctgggggatgacacaagcctggctctcacgagcaccctgatttctgttcctgacagagacccagcctcgcctttaaggatggcaaacgaattcgattataaggatgacgatgacaagctcgagcatcaccaccatcaccactaa

SEQ ID NO: 283 - protein, 122 aa, Artificial Sequence; identical to SEQ ID NO: 29

SEQ ID NO: 284 - DNA, 366 bp, Artificial Sequence
  source 1..366: mol_type = other DNA
caggtccagctgcagcagcctggggccgaaatcgtgagacctggcgctagcgtgaagctgtcttgcaaggccagcggctacaccttcacagacaactggatgggctgggtgaagcagagacctggccagggcctggagtggatcggcgccatcgatccctccgacagcttcaccaattacaatcagaactttaagggcaaggccaccctgacagtggatacctcttccagcacagcttacatgcagctgtctagcctgacaagcgaggattctgccgtgtatttttgtacaagaagcggctattacggcagccctaagctgggcggcgactactggggccagggcaccacactgacagtgtcttcc

SEQ ID NO: 285 - protein, 106 aa, Artificial Sequence; identical to SEQ ID NO: 31

SEQ ID NO: 286 - DNA, 318 bp, Artificial Sequence
  source 1..318: mol_type = other DNA
cagattgtgctgactcagtcacccgctatcatgtccgcttctctgggcgaggagatcacactgacctgttctgcctccagctctatctcctacatgcactggtatcagcagaagtctggcacctctccaaagctgctgatctactccacctctaacctggcttctggcgtgccttccagattctctggcagcggctctggcaccttctattccctgacaatctccagcgtggaggctgaggatgccgctgactactattgccaccagtggaactcttacccatgcacatttggcggcggcacaaagctggagatcaag

SEQ ID NO: 287 - protein, 8 aa, Artificial Sequence
GLSLTSIN

SEQ ID NO: 288 - DNA, 24 bp, Artificial Sequence
  source 1..24: mol_type = other DNA
ggcctttccctgacgagcatcaac

SEQ ID NO: 289 - protein, 7 aa, Artificial Sequence
IWSDGDT

SEQ ID NO: 290 - DNA, 21 bp, Artificial Sequence
  source 1..21: mol_type = other DNA
atttggagtgatggggatact

SEQ ID NO: 291 - protein, 6 aa, Artificial Sequence
ARGIRD

SEQ ID NO: 292 - DNA, 18 bp, Artificial Sequence
  source 1..18: mol_type = other DNA
gctagaggcataagggac

SEQ ID NO: 293 - protein, 11 aa, Artificial Sequence
QSLKYSDGKTY

SEQ ID NO: 294 - DNA, 33 bp, Artificial Sequence
  source 1..33: mol_type = other DNA
cagtccctgaagtatagcgatgggaaaacctac

SEQ ID NO: 295-296 - skipped (2 entries)

SEQ ID NO: 297 - protein, 9 aa, Artificial Sequence
CQGSYSPHT

SEQ ID NO: 298 - DNA, 27 bp, Artificial Sequence
  source 1..27: mol_type = other DNA
tgtcaagggtcctattcaccccatacc

SEQ ID NO: 299 - protein, 112 aa, Artificial Sequence
QVQLKASGPGLVQPSQTLSLTCTVSGLSLTSININWIRQPPGKGLEWMGVIWSDGDTDFNSAVKSRLSISRDTSKSQVFLNMNSLQTEDTAMYFCARGIRDWGQGVMVTVSS

SEQ ID NO: 300 - DNA, 336 bp, Artificial Sequence
  source 1..336: mol_type = other DNA
caggtccagctgaaagccagtggtcctggactggttcagccaagccagaccctctcactcacatgcaccgtttctggcctttccctgacgagcatcaacatcaattggattcggcaaccacctggcaaaggattggagtggatgggcgtgatttggagtgatggggatactgacttcaactccgctgtgaagtcccgactgtccatttcacgcgataccagcaagtctcaggtgttcctgaacatgaatagcctgcagactgaggacactgccatgtacttctgtgctagaggcataagggactggggtcaaggagtcatggttaccgtgtcatct

SEQ ID NO: 301 - protein, 112 aa, Artificial Sequence
DIVMTQTPLSLSVAIGQSASISCKSSQSLKYSDGKTYLNWVFQSPGQSPKRLIYQVSKLDSGVPDRFSGTGSETDFTLKISRVEAEDLGVYYCCQGSYSPHTFGSGTKLEIK

SEQ ID NO: 302 - DNA, 336 bp, Artificial Sequence
  source 1..336: mol_type = other DNA
gacatagtgatgacccagacacccttgagtctgagtgttgccattggccaaagtgcctctatctcctgcaagtcaagtcagtccctgaagtatagcgatgggaaaacctacctgaactgggtctttcagagcccaggtcagtcacccaaacggctgatttaccaggtcagcaaactcgactctggagtaccagaccgcttttccggaacaggtagcgagactgacttcaccctcaagatctctagggtggaagccgaggatcttggcgtgtattactgctgtcaagggtcctattcaccccatacctttggttccggcacaaagctggagatcaag